European Patent Application EP 4 446 363 A2, published October 16, 2024. Title: DERMAL FILLERS AND METHODS OF USE THEREOF. Applicant: CollPlant Ltd. Application EP, filed May 2, 2019. The sequence listing filed with the application follows.

SEQUENCE LISTING (45 sequences)

SEQ ID NO: 1 - DNA, 4662 bp, synthetic construct
  misc_feature 1..4662: note = Synthetic sequence containing the coding regions of the vacuolar signal sequence of barley gene for Thiol protease aleurain precursor fused to the human Collagen alpha 1(I) chain and flanking regions
  source 1..4662: mol_type = other DNA
gcgatgcatgtaatgtcatgagccacatgatccaatggccacaggaacgtaagaatgtagatagatttgattttgtccgttagatagcaaacaacattataaaaggtgtgtatcaatacgaactaattcactcattggattcatagaagtccattcctcctaagtatctaaaccatggctcacgctcgtgttctcctcctcgctctcgctgttttggcaacagctgctgtggctgtggcttctagttcttcttttgctgattcaaaccctattagacctgttactgatagagcagcttccactttggctcaattgcaagaggagggccaggttgagggccaagatgaggatatccctccaattacatgcgtgcaaaatggcttgcgttaccacgatagggatgtgtggaaacctgaaccttgtcgtatctgtgtgtgtgataacggcaaggtgctctgcgatgatgttatctgcgatgagacaaaaaattgccctggcgctgaagttcctgagggcgagtgttgccctgtgtgccctgatggttccgagtccccaactgatcaggaaactactggcgtggagggcccaaaaggagatactggtccacgtggtcctaggggtccagcaggtcctccaggtagagatggtattccaggccagcctggattgccaggaccaccaggcccacctggcccaccaggacctcctggtcttggtggaaatttcgctccacaactctcttatggctatgatgagaagtcaacaggtggtatttccgttccaggtcctatgggaccatccggaccaagaggtctcccaggtcctccaggtgctcctggacctcaaggctttcaaggacctccaggcgaaccaggagaaccaggcgcttctggaccaatgggcccaaggggaccacctggcccaccaggaaaaaatggcgatgatggcgaagctggaaagcctggtcgtcctggagagagaggtcctcctggcccacagggtgcaagaggcttgccaggaactgctggcttgcctggaatgaagggacataggggcttctccggcctcgatggcgctaagggtgatgctggccctgctggaccaaagggcgagccaggttcccctggagaaaacggtgctcctggacaaatgggtcctcgtggacttccaggagaaaggggtcgtccaggcgctccaggaccagcaggtgctaggggaaacgatggtgcaacaggcgctgctggccctcctggcccaactggtcctgctggccctccaggattcccaggcgcagttggagctaaaggagaagcaggaccacagggccctaggggttctgaaggacctcagggtgttagaggtgaaccaggtcctccaggcccagctggagcagctggtccagcaggaaatccaggtgctgatggtcaacctggagctaagggcgctaatggcgcaccaggtatcgcaggcgcaccaggttttcctggcgctagaggcccaagtggtcctcaaggaccaggtggaccaccaggtccaaaaggcaattctggcgaacctggcgctccaggttctaaaggagatactggtgctaaaggcgaaccaggacctgttggtgttcagggtcctcctggtcctgctggagaagaaggaaaaagaggtgctcgtggagaaccaggaccaactggacttcctggacctcctggtgaacgtggcggacctggctcaaggggtttccctggagctgatggagtggcaggtccaaaaggccctgctggagagagaggttcaccaggtccagctggtcctaagggctcccctggtgaagcaggtagaccaggcgaagcaggattgccaggcgcaaagggattgacaggctctcctggtagtcctggcccagatggaaaaacaggcccaccaggtccagcaggacaagatggacgtccaggcccaccaggtcctcctggagcaaggggacaagctggcgttatgggttttccaggacctaaaggtgctgctggagagccaggaaaggcaggtgaaagaggagttcctggtccaccaggagcagtgggtcctgctggcaaagatggtgaagctggagcacagggccctccaggccctgctggcccagctggcgaacgtggagaacaaggcccagctggtagtccaggatttcaaggattgcctggccctgctggccctccaggagaagcaggaaaacctggagaacaaggagttcctggtgatttgggagcacctggaccttcaggagcacgtggtgaaagaggcttccctggcgagaggggtgttcaaggtccaccaggtccagcaggacctagaggtgctaatggcgctcctggcaacgatggagcaaaaggtgatgctggtgctcctggcgcacctggaagtcagggtgctcctggattgcaaggaatgcctggagagaggggtgctgctggcttgccaggcccaaagggcgataggggtgatgctggaccaaaaggtgctgatggatccccaggaaaagatggagttcgtggtcttactggcccaatcggacctccaggccctgctggcgctccaggtgataagggcgaaagtggcccaagtggacctgctggacctactggtgctagaggtgcacctggtgataggggtgaacctggaccacctggtccagctggttttgctggtcctcctggagctgatggacaacctggcgcaaagggtgaaccaggtgatgctggcgcaaagggagatgctggtccacctggacctgctggtccagcaggcccccctgggccaatcggtaatgttggagcaccaggtgctaagggagctaggggttccgctggtccacctggagcaacaggatttccaggcgctgctggtagagttggcccaccaggcccatccggaaacgcaggccctcctggtcctccaggtcctgctggcaaggagggtggcaaaggaccaaggggcgaaactggccctgctggtagacctggcgaagttggccctcctggaccaccaggtccagcaggagaaaaaggttccccaggagctgatggcccagctggtgctccaggaactccaggccctcaaggtattgctggacagagaggcgttgtgggactccctggtcaaaggggagagagaggatttccaggcttgccaggacctagtggagaacctggaaaacaaggcccatcaggcgctagtggagagcgtggacctcctggccctatgggacctcctggattggctggcccacctggcgaatcaggtcgtgaaggcgcaccaggcgcagaaggatcacctggaagagatggatcccctggtgctaaaggcgatcgtggagaaactggtccagcaggcccaccaggcgcaccaggtgcacctggcgctccaggacctgtgggaccagctggaaaatccggagataggggcgagacaggcccagcaggaccagctggacctgttggccctgctggcgctcgtggaccagcaggacctcaaggaccaaggggagataagggagaaacaggcgaacaaggcgataggggcattaagggtcataggggttttagtggcctccagggtcctcctggcccacctggatcaccaggagaacagggaccatctggtgcttccggcccagctggtccaagaggacctccaggatcagctggtgcacctggaaaagatggtcttaacggtctcccaggaccaatcggccctccaggacctagaggaagaacaggagatgctggccctgttggccctccaggacctcctggtccaccaggtccacctggtcctccatcagctggattcgatttttcatttcttccacagccaccacaagagaaagctcacgatggcggcagatattaccgtgctgatgatgctaacgttgttagggatagagatttggaagtggatacaactttgaaatccctctcccagcaaattgaaaacattagatctccagaaggttcacgtaaaaacccagctagaacatgtcgtgatttgaaaatgtgtcactccgattggaaaagtggtgaatactggattgatccaaatcagggctgtaatctcgatgctatcaaagttttctgtaacatggaaacaggcgaaacatgcgtttatcctactcaaccttccgtggctcagaaaaattggtacatctcaaaaaatcctaaagataagaggcacgtttggttcggtgaaagtatgactgatggatttcaatttgagtacggcggtcaaggtagtgatccagctgatgtggctattcaactcacatttttgcgtcttatgtccacagaggcatcacaaaacatcacttaccactgcaaaaacagtgtggcttatatggatcaacaaacaggaaaccttaagaaggctcttcttttgaagggctcaaacgagattgagattagagcagagggcaactcaaggtttacttattcagttactgttgatggctgcacttcacatactggcgcttggggtaaaacagttatcgagtataagactacaaaaacatcaagactcccaatcattgatgttgctcctctcgatgttggcgctcctgatcaagagttcggttttgatgtgggcccagtttgtttcctctaatgagctcgcggccgcatc

SEQ ID NO: 2 - DNA, 4662 bp, synthetic construct; identical to SEQ ID NO: 1
  misc_feature 1..4662: note = Synthetic sequence of the vacuolar signal sequence of barley gene for Thiol protease aleurain precursor fused to the human Collagen alpha 1(I) chain and flanking regions
  source 1..4662: mol_type = other DNA
  CDS 175..4644: protein_id = 43; translation = MAHARVLLLALAVLATAAVAVASSSSFADSNPIRPVTDRAASTLAQLQEEGQVEGQDEDIPPITCVQNGLRYHDRDVWKPEPCRICVCDNGKVLCDDVICDETKNCPGAEVPEGECCPVCPDGSESPTDQETTGVEGPKGDTGPRGPRGPAGPPGRDGIPGQPGLPGPPGPPGPPGPPGLGGNFAPQLSYGYDEKSTGGISVPGPMGPSGPRGLPGPPGAPGPQGFQGPPGEPGEPGASGPMGPRGPPGPPGKNGDDGEAGKPGRPGERGPPGPQGARGLPGTAGLPGMKGHRGFSGLDGAKGDAGPAGPKGEPGSPGENGAPGQMGPRGLPGERGRPGAPGPAGARGNDGATGAAGPPGPTGPAGPPGFPGAVGAKGEAGPQGPRGSEGPQGVRGEPGPPGPAGAAGPAGNPGADGQPGAKGANGAPGIAGAPGFPGARGPSGPQGPGGPPGPKGNSGEPGAPGSKGDTGAKGEPGPVGVQGPPGPAGEEGKRGARGEPGPTGLPGPPGERGGPGSRGFPGADGVAGPKGPAGERGSPGPAGPKGSPGEAGRPGEAGLPGAKGLTGSPGSPGPDGKTGPPGPAGQDGRPGPPGPPGARGQAGVMGFPGPKGAAGEPGKAGERGVPGPPGAVGPAGKDGEAGAQGPPGPAGPAGERGEQGPAGSPGFQGLPGPAGPPGEAGKPGEQGVPGDLGAPGPSGARGERGFPGERGVQGPPGPAGPRGANGAPGNDGAKGDAGAPGAPGSQGAPGLQGMPGERGAAGLPGPKGDRGDAGPKGADGSPGKDGVRGLTGPIGPPGPAGAPGDKGESGPSGPAGPTGARGAPGDRGEPGPPGPAGFAGPPGADGQPGAKGEPGDAGAKGDAGPPGPAGPAGPPGPIGNVGAPGAKGARGSAGPPGATGFPGAAGRVGPPGPSGNAGPPGPPGPAGKEGGKGPRGETGPAGRPGEVGPPGPPGPAGEKGSPGADGPAGAPGTPGPQGIAGQRGVVGLPGQRGERGFPGLPGPSGEPGKQGPSGASGERGPPGPMGPPGLAGPPGESGREGAPGAEGSPGRDGSPGAKGDRGETGPAGPPGAPGAPGAPGPVGPAGKSGDRGETGPAGPAGPVGPAGARGPAGPQGPRGDKGETGEQGDRGIKGHRGFSGLQGPPGPPGSPGEQGPSGASGPAGPRGPPGSAGAPGKDGLNGLPGPIGPPGPRGRTGDAGPVGPPGPPGPPGPPGPPSAGFDFSFLPQPPQEKAHDGGRYYRADDANVVRDRDLEVDTTLKSLSQQIENIRSPEGSRKNPARTCRDLKMCHSDWKSGEYWIDPNQGCNLDAIKVFCNMETGETCVYPTQPSVAQKNWYISKNPKDKRHVWFGESMTDGFQFEYGGQGSDPADVAIQLTFLRLMSTEASQNITYHCKNSVAYMDQQTGNLKKALLLKGSNEIEIRAEGNSRFTYSVTVDGCTSHTGAWGKTVIEYKTTKTSRLPIIDVAPLDVGAPDQEFGFDVGPVCFL

SEQ ID NO: 3 - protein, 1489 aa, synthetic construct
  REGION 1..1489: note = Synthetic Construct
MAHARVLLLALAVLATAAVAVASSSSFADSNPIRPVTDRAASTLAQLQEEGQVEGQDEDIPPITCVQNGLRYHDRDVWKPEPCRICVCDNGKVLCDDVICDETKNCPGAEVPEGECCPVCPDGSESPTDQETTGVEGPKGDTGPRGPRGPAGPPGRDGIPGQPGLPGPPGPPGPPGPPGLGGNFAPQLSYGYDEKSTGGISVPGPMGPSGPRGLPGPPGAPGPQGFQGPPGEPGEPGASGPMGPRGPPGPPGKNGDDGEAGKPGRPGERGPPGPQGARGLPGTAGLPGMKGHRGFSGLDGAKGDAGPAGPKGEPGSPGENGAPGQMGPRGLPGERGRPGAPGPAGARGNDGATGAAGPPGPTGPAGPPGFPGAVGAKGEAGPQGPRGSEGPQGVRGEPGPPGPAGAAGPAGNPGADGQPGAKGANGAPGIAGAPGFPGARGPSGPQGPGGPPGPKGNSGEPGAPGSKGDTGAKGEPGPVGVQGPPGPAGEEGKRGARGEPGPTGLPGPPGERGGPGSRGFPGADGVAGPKGPAGERGSPGPAGPKGSPGEAGRPGEAGLPGAKGLTGSPGSPGPDGKTGPPGPAGQDGRPGPPGPPGARGQAGVMGFPGPKGAAGEPGKAGERGVPGPPGAVGPAGKDGEAGAQGPPGPAGPAGERGEQGPAGSPGFQGLPGPAGPPGEAGKPGEQGVPGDLGAPGPSGARGERGFPGERGVQGPPGPAGPRGANGAPGNDGAKGDAGAPGAPGSQGAPGLQGMPGERGAAGLPGPKGDRGDAGPKGADGSPGKDGVRGLTGPIGPPGPAGAPGDKGESGPSGPAGPTGARGAPGDRGEPGPPGPAGFAGPPGADGQPGAKGEPGDAGAKGDAGPPGPAGPAGPPGPIGNVGAPGAKGARGSAGPPGATGFPGAAGRVGPPGPSGNAGPPGPPGPAGKEGGKGPRGETGPAGRPGEVGPPGPPGPAGEKGSPGADGPAGAPGTPGPQGIAGQRGVVGLPGQRGERGFPGLPGPSGEPGKQGPSGASGERGPPGPMGPPGLAGPPGESGREGAPGAEGSPGRDGSPGAKGDRGETGPAGPPGAPGAPGAPGPVGPAGKSGDRGETGPAGPAGPVGPAGARGPAGPQGPRGDKGETGEQGDRGIKGHRGFSGLQGPPGPPGSPGEQGPSGASGPAGPRGPPGSAGAPGKDGLNGLPGPIGPPGPRGRTGDAGPVGPPGPPGPPGPPGPPSAGFDFSFLPQPPQEKAHDGGRYYRADDANVVRDRDLEVDTTLKSLSQQIENIRSPEGSRKNPARTCRDLKMCHSDWKSGEYWIDPNQGCNLDAIKVFCNMETGETCVYPTQPSVAQKNWYISKNPKDKRHVWFGESMTDGFQFEYGGQGSDPADVAIQLTFLRLMSTEASQNITYHCKNSVAYMDQQTGNLKKALLLKGSNEIEIRAEGNSRFTYSVTVDGCTSHTGAWGKTVIEYKTTKTSRLPIIDVAPLDVGAPDQEFGFDVGPVCFL

SEQ ID NO: 4 - DNA, 4362 bp, synthetic construct
  misc_feature 1..4362: note = Synthetic sequence containing the coding regions of the vacuolar signal sequence of barley gene for Thiol protease aleurain precursor fused to the human Collagen alpha 2(I) chain and flanking regions
  source 1..4362: mol_type = other DNA
gcgatgcatgtaatgtcatgagccacatgatccaatggccacaggaacgtaagaatgtagatagatttgattttgtccgttagatagcaaacaacattataaaaggtgtgtatcaatacgaactaattcactcattggattcatagaagtccattcctcctaagtatctaaaccatggctcacgctcgtgttctcctcctcgctctcgctgttttggcaacagctgctgtggctgtggcttcaagttctagttttgctgattccaacccaattcgtccagttactgatagagcagcttccactttggctcaattgcttcaagaagaaactgtgaggaagggccctgctggcgataggggccctaggggcgaaaggggtccaccaggacctccaggcagggatggcgaagatggtccaactggccctcctggacctcctggccctccagggccacccggcttgggcggaaacttcgcagctcaatacgatggcaagggtgttggtcttggtcctggtcctatgggcttgatgggacctagaggcccacctggtgctgctggtgctcctggaccacagggttttcagggaccagctggcgagccaggagagccaggccaaacaggaccagctggtgcaaggggacctgctggacctcctggaaaagctggtgaagatggtcacccaggcaaaccaggacgtcctggcgaaagaggtgttgttggaccacaaggcgctaggggatttccaggtacacctggattgccaggttttaagggcattcgtggtcataacggcctcgatggattgaagggacagcctggcgcacctggcgttaagggtgaacctggagcaccaggtgaaaacggtactcctggccagactggtgcaagaggactcccaggtgaaaggggtagagttggtgctcctggacctgctggagctaggggtagtgatggtagtgttggtcctgtgggccctgctggtccaatcggttccgctggcccacctggattcccaggcgctccaggacctaaaggagaaatcggtgctgtgggtaacgcaggtcctactggtccagcaggtcctcgtggagaagtgggattgccaggactttctggtccagtgggccctccaggcaaccctggagctaacggcttgacaggagctaaaggcgcagcaggactccctggagtggctggcgcaccaggattgcctggtccaaggggtatcccaggccctgttggcgcagctggagctactggtgcacgtggacttgttggcgaaccaggccctgctggatcaaaaggcgagtctggaaataagggagaacctggttctgctggacctcaaggtcctcctggaccttctggagaagaaggaaaaaggggaccaaatggcgaggctggatcagcaggtccaccaggaccacctggacttcgtggatcccctggtagtagaggacttccaggcgctgatggtagagcaggcgttatgggaccaccaggaagtagaggagcatccggtccagcaggagttaggggtcctaacggagatgctggtagaccaggtgaaccaggtcttatgggcccaaggggcctcccaggtagtccaggaaatatcggccctgctggaaaagaaggccctgttggacttccaggtattgatggacgtcctggccctattggcccagcaggtgcaagaggagaacctggcaatattggatttccaggaccaaagggtccaacaggcgatcctggaaaaaatggagataagggtcatgctggattggcaggcgcaaggggcgctcctggtccagatggaaacaacggcgcacagggtccacctggccctcagggtgttcaaggcggaaaaggcgaacaaggcccagctggaccaccaggctttcaaggcttgccaggaccaagtggtccagcaggtgaagttggcaagccaggcgagcgtggacttcatggcgagtttggactccctggaccagcaggaccaaggggtgaaagaggccctcctggagagagtggcgctgctggaccaacaggcccaatcggtagtagaggtcctagtggacctccaggcccagatggaaataagggtgaaccaggagttgtgggcgctgttggaacagctggtccttcaggaccatcaggactcccaggcgagagaggcgctgctggcattcctggaggaaaaggtgaaaaaggcgaacctggcctccgtggcgaaatcggaaatcctggacgtgatggtgctcgtggtgcacacggcgctgtgggcgctccaggccctgctggtgctactggtgatagaggagaggctggcgcagctggcccagcaggtcctgctggcccaaggggtagtcctggtgaaagaggcgaagttggacctgctggccctaacggctttgctggccctgctggagcagcaggtcaacctggcgctaaaggtgaaaggggcggaaagggcccaaaaggtgaaaatggcgttgtgggaccaactggtccagtgggcgcagctggacctgctggtccaaatggaccaccaggaccagcaggtagtagaggagatggtggacctccaggaatgacaggttttccaggtgctgctggtagaacaggacctcctggtcctagtggtatttctggtccaccaggaccaccaggtcctgctggaaaagaaggattgaggggtccacgtggtgatcaaggaccagtgggcagaactggtgaagttggcgcagtgggaccacctggttttgctggagaaaagggcccttctggagaggcaggaacagctggtcctcctggtacacctggacctcaaggacttttgggtgcacctggtattctcggattgccaggaagtaggggcgaacgtggacttcctggcgtggcaggagcagttggagaacctggccctctcggaatcgcaggcccaccaggcgcaagaggaccaccaggagctgttggatcaccaggcgtgaatggtgcacctggcgaggctggtcgtgatggaaacccaggaaatgatggcccaccaggaagagatggtcaacctggacacaaaggcgagaggggctacccaggaaatattggcccagttggtgctgctggcgcaccaggcccacacggtccagttggaccagcaggaaaacacggtaatcgtggcgaaacaggcccttcaggcccagtgggacctgctggtgctgttggcccaagaggaccatctggacctcaaggcattagaggcgataagggagagcctggcgaaaaaggacctagaggcttgcctggttttaaaggacacaacggtctccaaggacttccaggtatcgctggtcatcatggagatcagggtgctcctggatcagtgggtccagcaggtcctagaggcccagcaggcccttccggtccagcaggaaaggatggacgtactggccaccctggaactgtgggccctgctggaattagaggtcctcaaggtcatcagggccctgctggccctccaggtccaccaggtcctccaggcccaccaggagtttcaggtggtggttacgattttggttacgatggtgatttttaccgtgctgatcaacctagaagtgctccttctctccgtcctaaagattatgaagttgatgctactttgaaatcacttaacaaccagattgagactcttctcacacctgagggatcaagaaagaatccagcacgtacatgccgtgatctcagacttagtcacccagagtggtcaagtggctattattggattgatcctaatcagggttgtacaatggaggctatcaaagtttactgtgattttccaactggagagacatgtattagggcacaacctgagaacattccagctaaaaattggtatcgttcctctaaagataagaaacatgtttggctcggagagactattaacgctggttctcagttcgagtataatgttgagggcgttacttctaaagagatggcaactcagctcgcttttatgagattgctcgctaactacgcatcccaaaacatcacttatcactgcaaaaattccattgcatatatggatgaggagacaggaaatttgaagaaagcagttattctccaaggtagtaacgatgttgagcttgtggctgagggaaatagtagattcacttacacagttttggtggatggatgctcaaagaaaactaatgagtggggcaagacaatcattgagtacaagacaaataagccttctaggctcccatttctcgatattgcacctcttgatatcggaggagctgatcacgagttttttgttgatatcggacctgtttgttttaagtaatgagctcgcggccgcatc

SEQ ID NO: 5 - DNA, 4362 bp, synthetic construct; identical to SEQ ID NO: 4
  misc_feature 1..4362: note = Synthetic sequence of the vacuolar signal sequence of barley gene for Thiol protease aleurain precursor fused to the human Collagen alpha 2(I) chain and flanking regions
  source 1..4362: mol_type = other DNA
  CDS 175..4344: protein_id = 44; translation = MAHARVLLLALAVLATAAVAVASSSSFADSNPIRPVTDRAASTLAQLLQEETVRKGPAGDRGPRGERGPPGPPGRDGEDGPTGPPGPPGPPGPPGLGGNFAAQYDGKGVGLGPGPMGLMGPRGPPGAAGAPGPQGFQGPAGEPGEPGQTGPAGARGPAGPPGKAGEDGHPGKPGRPGERGVVGPQGARGFPGTPGLPGFKGIRGHNGLDGLKGQPGAPGVKGEPGAPGENGTPGQTGARGLPGERGRVGAPGPAGARGSDGSVGPVGPAGPIGSAGPPGFPGAPGPKGEIGAVGNAGPTGPAGPRGEVGLPGLSGPVGPPGNPGANGLTGAKGAAGLPGVAGAPGLPGPRGIPGPVGAAGATGARGLVGEPGPAGSKGESGNKGEPGSAGPQGPPGPSGEEGKRGPNGEAGSAGPPGPPGLRGSPGSRGLPGADGRAGVMGPPGSRGASGPAGVRGPNGDAGRPGEPGLMGPRGLPGSPGNIGPAGKEGPVGLPGIDGRPGPIGPAGARGEPGNIGFPGPKGPTGDPGKNGDKGHAGLAGARGAPGPDGNNGAQGPPGPQGVQGGKGEQGPAGPPGFQGLPGPSGPAGEVGKPGERGLHGEFGLPGPAGPRGERGPPGESGAAGPTGPIGSRGPSGPPGPDGNKGEPGVVGAVGTAGPSGPSGLPGERGAAGIPGGKGEKGEPGLRGEIGNPGRDGARGAHGAVGAPGPAGATGDRGEAGAAGPAGPAGPRGSPGERGEVGPAGPNGFAGPAGAAGQPGAKGERGGKGPKGENGVVGPTGPVGAAGPAGPNGPPGPAGSRGDGGPPGMTGFPGAAGRTGPPGPSGISGPPGPPGPAGKEGLRGPRGDQGPVGRTGEVGAVGPPGFAGEKGPSGEAGTAGPPGTPGPQGLLGAPGILGLPGSRGERGLPGVAGAVGEPGPLGIAGPPGARGPPGAVGSPGVNGAPGEAGRDGNPGNDGPPGRDGQPGHKGERGYPGNIGPVGAAGAPGPHGPVGPAGKHGNRGETGPSGPVGPAGAVGPRGPSGPQGIRGDKGEPGEKGPRGLPGFKGHNGLQGLPGIAGHHGDQGAPGSVGPAGPRGPAGPSGPAGKDGRTGHPGTVGPAGIRGPQGHQGPAGPPGPPGPPGPPGVSGGGYDFGYDGDFYRADQPRSAPSLRPKDYEVDATLKSLNNQIETLLTPEGSRKNPARTCRDLRLSHPEWSSGYYWIDPNQGCTMEAIKVYCDFPTGETCIRAQPENIPAKNWYRSSKDKKHVWLGETINAGSQFEYNVEGVTSKEMATQLAFMRLLANYASQNITYHCKNSIAYMDEETGNLKKAVILQGSNDVELVAEGNSRFTYTVLVDGCSKKTNEWGKTIIEYKTNKPSRLPFLDIAPLDIGGADHEFFVDIGPVCFK

SEQ ID NO: 6 - protein, 1389 aa, synthetic construct
  REGION 1..1389: note = Synthetic Construct
MAHARVLLLALAVLATAAVAVASSSSFADSNPIRPVTDRAASTLAQLLQEETVRKGPAGDRGPRGERGPPGPPGRDGEDGPTGPPGPPGPPGPPGLGGNFAAQYDGKGVGLGPGPMGLMGPRGPPGAAGAPGPQGFQGPAGEPGEPGQTGPAGARGPAGPPGKAGEDGHPGKPGRPGERGVVGPQGARGFPGTPGLPGFKGIRGHNGLDGLKGQPGAPGVKGEPGAPGENGTPGQTGARGLPGERGRVGAPGPAGARGSDGSVGPVGPAGPIGSAGPPGFPGAPGPKGEIGAVGNAGPTGPAGPRGEVGLPGLSGPVGPPGNPGANGLTGAKGAAGLPGVAGAPGLPGPRGIPGPVGAAGATGARGLVGEPGPAGSKGESGNKGEPGSAGPQGPPGPSGEEGKRGPNGEAGSAGPPGPPGLRGSPGSRGLPGADGRAGVMGPPGSRGASGPAGVRGPNGDAGRPGEPGLMGPRGLPGSPGNIGPAGKEGPVGLPGIDGRPGPIGPAGARGEPGNIGFPGPKGPTGDPGKNGDKGHAGLAGARGAPGPDGNNGAQGPPGPQGVQGGKGEQGPAGPPGFQGLPGPSGPAGEVGKPGERGLHGEFGLPGPAGPRGERGPPGESGAAGPTGPIGSRGPSGPPGPDGNKGEPGVVGAVGTAGPSGPSGLPGERGAAGIPGGKGEKGEPGLRGEIGNPGRDGARGAHGAVGAPGPAGATGDRGEAGAAGPAGPAGPRGSPGERGEVGPAGPNGFAGPAGAAGQPGAKGERGGKGPKGENGVVGPTGPVGAAGPAGPNGPPGPAGSRGDGGPPGMTGFPGAAGRTGPPGPSGISGPPGPPGPAGKEGLRGPRGDQGPVGRTGEVGAVGPPGFAGEKGPSGEAGTAGPPGTPGPQGLLGAPGILGLPGSRGERGLPGVAGAVGEPGPLGIAGPPGARGPPGAVGSPGVNGAPGEAGRDGNPGNDGPPGRDGQPGHKGERGYPGNIGPVGAAGAPGPHGPVGPAGKHGNRGETGPSGPVGPAGAVGPRGPSGPQGIRGDKGEPGEKGPRGLPGFKGHNGLQGLPGIAGHHGDQGAPGSVGPAGPRGPAGPSGPAGKDGRTGHPGTVGPAGIRGPQGHQGPAGPPGPPGPPGPPGVSGGGYDFGYDGDFYRADQPRSAPSLRPKDYEVDATLKSLNNQIETLLTPEGSRKNPARTCRDLRLSHPEWSSGYYWIDPNQGCTMEAIKVYCDFPTGETCIRAQPENIPAKNWYRSSKDKKHVWLGETINAGSQFEYNVEGVTSKEMATQLAFMRLLANYASQNITYHCKNSIAYMDEETGNLKKAVILQGSNDVELVAEGNSRFTYTVLVDGCSKKTNEWGKTIIEYKTNKPSRLPFLDIAPLDIGGADHEFFVDIGPVCFK

SEQ ID NO: 7 - DNA, 127 bp, synthetic construct
  misc_feature 1..127: note = Synthetic sequence containing the coding region of the appoplast signal of Arabidopsis thaliana endo-1,4-beta-glucanase and flanking regions
  source 1..127: mol_type = other DNA
gccatggctaggaagtctttgattttcccagtgattcttcttgctgtgcttcttttctctccacctatttactctgctggacacgattatagggatgctcttaggaagtcatctatggctcaattgc

SEQ ID NO: 8 - DNA, 127 bp, synthetic construct; identical to SEQ ID NO: 7
  misc_feature 1..127: note = Synthetic sequence of the appoplast signal of Arabidopsis thaliana endo-1,4-beta-glucanase and flanking regions
  source 1..127: mol_type = other DNA
  CDS 10..120: protein_id = 45; translation = RKSLIFPVILLAVLLFSPPIYSAGHDYRDALRKSSMA

SEQ ID NO: 9 - protein, 37 aa, synthetic construct
  REGION 1..37: note = Synthetic Construct
RKSLIFPVILLAVLLFSPPIYSAGHDYRDALRKSSMA

SEQ ID NO: 10 - DNA, 1037 bp, synthetic construct
  misc_feature 1..1037: note = Chrysanthemum rbcS1 promoter and 5' UTR
  source 1..1037: mol_type = other DNA
aaatggcgcgccaagcttagacaaacaccccttgttatacaaagaatttcgctttacaaaatcaaattcgagaaaataatatatgcactaaataagatcattcggatccaatctaaccaattacgatacgctttgggtacacttgatttttgtttcagtagttacatatatcttgttttatatgctatctttaaggatcttcactcaaagactatttgttgatgttcttgatggggctcggaagatttgatatgatacactctaatctttaggagataccagccaggattatattcagtaagacaatcaaattttacgtgttcaaactcgttatcttttcatttaatggatgagccagaatctctatagaatgattgcaatcgagaatatgttcggccgatatccctttgttggcttcaatattctacatatcacacaagaatcgaccgtattgtaccctctttccataaaggaacacacagtatgcagatgcttttttcccacatgcagtaacataggtattcaaaaatggctaaaagaagttggataacaaattgacaactatttccatttctgttatataaatttcacaacacacaaaagcccgtaatcaagagtctgcccatgtacgaaataacttctattatttggtattgggcctaagcccagctcagagtacgtgggggtaccacatataggaaggtaacaaaatactgcaagatagccccataacgtaccagcctctccttaccacgaagagataagatataagacccaccctgccacgtgtcacatcgtcatggtggttaatgataagggattacatccttctatgtttgtggacatgatgcatgtaatgtcatgagccacatgatccaatggccacaggaacgtaagaatgtagatagatttgattttgtccgttagatagcaaacaacattataaaaggtgtgtatcaatacgaactaattcactcattggattcatagaagtccattcctcctaagtatctaaacatatgcaattgtcgactaaa

SEQ ID NO: 11 - DNA, 975 bp, synthetic construct
  misc_feature 1..975: note = Chrysanthemum rbcS1 3'UTR and terminator
  source 1..975: mol_type = other DNA
aaaaggatccgcggccgcataagttttactatttaccaagacttttgaatattaaccttcttgtaacgagtcggttaaatttgattgtttagggttttgtattatttttttttggtcttttaattcatcactttaattccctaattgtctgttcatttcgttgtttgtttccggatcgataatgaaatgtaagagatatcatatataaataataaattgtcgtttcatatttgcaatctttttttacaaacctttaattaattgtatgtatgacattttcttcttgttatattagggggaaataatgttaaataaaagtacaaaataaactacagtacatcgtactgaataaattacctagccaaaaagtacacctttccatatacttcctacatgaaggcattttcaacattttcaaataaggaatgctacaaccgcataataacatccacaaatttttttataaaataacatgtcagacagtgattgaaagattttattatagtttcgttatcttcttttctcattaagcgaatcactacctaacacgtcattttgtgaaatattttttgaatgtttttatatagttgtagcattcctcttttcaaattagggtttgtttgagatagcatttcagccggttcatacaacttaaaagcatactctaatgctggaaaaaagactaaaaaatcttgtaagttagcgcagaatattgacccaaattatatacacacatgaccccatatagagactaattacacttttaaccactaataattattactgtattataacatctactaattaaacttgtgagtttttgctagaattattatcatatatactaaaaggcaggaacgcaaacattgccccggtactgtagcaactacggtagacgcattaattgtctatagtggacgcattaattaaccaaaaccgcctctttccccttcttcttgaagcttgagctctttt

SEQ ID NO: 12 - DNA, 1633 bp, synthetic construct
  misc_feature 1..1633: note = Synthetic sequence containing the coding regions of the vacuolar signal sequence of barley gene for Thiol protease aleurain precursor fused to the human Prolyl 4-hydroxylase beta subunit and flanking regions
  source 1..1633: mol_type = other DNA
ctcgagtaaaccatggctcatgctagggttttgcttttggctcttgctgttcttgctactgctgctgttgctgtggcttcttcttcatctttcgctgattctaacccaattaggccagtgactgatagagctgcttctactcttgctcaattggtcgacatggatgctccagaagaggaggatcacgttcttgtgcttaggaagtctaacttcgctgaagctcttgctgctcacaagtaccttcttgtggagttttatgctccttggtgcggacattgcaaagctcttgctccagagtatgctaaggctgctggaaagttgaaggctgagggatctgaaattaggcttgctaaagtggatgctactgaggagtctgatcttgctcaacagtacggagttaggggatacccaactattaagttcttcaggaacggagatactgcttctccaaaggagtatactgctggaagggaggctgatgatattgtgaactggcttaagaagagaactggaccagctgctactactcttccagatggagctgctgctgaatctcttgtggagtcatctgaggtggcagtgattggattcttcaaggatgtggagtctgattctgctaagcagttccttcaagctgctgaggctattgatgatattccattcggaattacttctaactctgatgtgttctctaagtaccagcttgataaggatggagtggtgcttttcaagaaattcgatgagggaaggaacaatttcgagggagaggtgacaaaggagaaccttcttgatttcattaagcacaaccagcttccacttgtgattgagttcactgagcagactgctccaaagattttcggaggagagattaagactcacattcttcttttccttccaaagtctgtgtctgattacgatggaaagttgtctaacttcaagactgctgctgagtctttcaagggaaagattcttttcattttcattgattctgatcacactgataaccagaggattcttgagttcttcggacttaagaaggaagagtgcccagctgttaggcttattactcttgaggaggagatgactaagtacaagccagagtctgaagaacttactgctgagaggattactgagttctgccacagattccttgagggaaagattaagccacaccttatgtctcaagagcttccagaggattgggataagcagccagttaaggtgttggtgggtaaaaacttcgaggatgtggctttcgatgagaagaagaacgtgttcgtggagttctacgcaccttggtgtggtcactgtaagcagcttgctccaatttgggataagttgggagagacttacaaggatcacgagaacattgtgattgctaagatggattctactgctaacgaggtggaggctgttaaggttcactctttcccaactttgaagttcttcccagcttctgctgataggactgtgattgattacaacggagaaaggactcttgatggattcaagaagttccttgagtctggaggacaagatggagctggagatgatgatgatcttgaggatttggaagaagctgaggagccagatatggaggaggatgatgatcagaaggctgtgtgatgagctc

SEQ ID NO: 13 - protein, 537 aa, synthetic construct
  REGION 1..537: note = Synthetic sequence containing the vacuolar signal sequence of barley gene for Thiol protease aleurain precursor fused to the human Prolyl 4-hydroxylase beta subunit and flanking regions
MAHARVLLLALAVLATAAVAVASSSSFADSNPIRPVTDRAASTLAQLVDMDAPEEEDHVLVLRKSNFAEALAAHKYLLVEFYAPWCGHCKALAPEYAKAAGKLKAEGSEIRLAKVDATEESDLAQQYGVRGYPTIKFFRNGDTASPKEYTAGREADDIVNWLKKRTGPAATTLPDGAAAESLVESSEVAVIGFFKDVESDSAKQFLQAAEAIDDIPFGITSNSDVFSKYQLDKDGVVLFKKFDEGRNNFEGEVTKENLLDFIKHNQLPLVIEFTEQTAPKIFGGEIKTHILLFLPKSVSDYDGKLSNFKTAAESFKGKILFIFIDSDHTDNQRILEFFGLKKEECPAVRLITLEEEMTKYKPESEELTAERITEFCHRFLEGKIKPHLMSQELPEDWDKQPVKVLVGKNFEDVAFDEKKNVFVEFYAPWCGHCKQLAPIWDKLGETYKDHENIVIAKMDSTANEVEAVKVHSFPTLKFFPASADRTVIDYNGERTLDGFKKFLESGGQDGAGDDDDLEDLEEAEEPDMEEDDDQKAV

SEQ ID NO: 14 - DNA, 1723 bp, synthetic construct
  misc_feature 1..1723: note = Synthetic sequence containing the coding regions of the vacuolar signal sequence of barley gene for Thiol protease aleurain precursor fused to the human Prolyl 4-hydroxylase alpha-1 subunit and flanking regions
  source 1..1723: mol_type = other DNA
ctcgagtaaaccatggctcatgctagggttttgcttttggctcttgctgttcttgctactgctgctgttgctgtggcttcttcttcatctttcgctgattctaacccaattaggccagtgactgatagagctgcttctactcttgctcaattggtcgacatgcacccaggattcttcacttctattggacagatgactgatcttattcacactgagaaggatcttgtgacttctcttaaggattacattaaggctgaggaggataagttggagcagattaagaagtgggctgagaagttggataggcttacttctactgctacaaaagatccagagggattcgttggtcatccagtgaacgctttcaagttgatgaagaggcttaacactgagtggagtgagcttgagaaccttgtgcttaaggatatgtctgatggattcatttctaaccttactattcagaggcagtacttcccaaatgatgaggatcaagtgggagctgctaaggctcttcttaggcttcaggatacttacaaccttgatactgatacaatttctaagggaaaccttccaggagttaagcacaagtctttccttactgctgaggattgcttcgagcttggaaaggttgcatacactgaggctgattactaccacactgagctttggatggaacaagctcttaggcaacttgatgagggagagatttctactattgataaggtgtcagtgcttgattacctttcttacgctgtgtaccagcagggtgatcttgataaggctcttttgcttactaagaagttgcttgagcttgatccagaacatcagagggctaacggaaaccttaagtacttcgagtacattatggctaaggaaaaggatgtgaacaagtctgcttctgatgatcagtctgatcaaaagactactccaaagaagaagggagtggctgttgattatcttcctgagaggcagaagtatgagatgttgtgtaggggagagggtattaagatgactccaaggaggcagaagaagttgttctgcaggtatcacgatggaaacaggaacccaaagttcattcttgctccagctaagcaagaagatgagtgggataagccaaggattattaggttccacgatattatttctgatgctgagattgagattgtgaaggatcttgctaagccaagacttaggagggctactatttctaaccctattactggtgatcttgagactgtgcactacaggatttctaagtctgcttggctttctggatacgagaacccagtggtgtctaggattaacatgaggattcaggatcttactggacttgatgtgtctactgctgaggagcttcaagttgctaactacggagttggaggacaatatgagccacacttcgatttcgctaggaaggatgagccagatgcttttaaggagcttggaactggaaacaggattgctacttggcttttctacatgtctgatgtttctgctggaggagctactgttttcccagaagtgggagcttctgtttggccaaagaagggaactgctgtgttctggtacaaccttttcgcttctggagagggagattactctactaggcatgctgcttgcccagttcttgttggaaacaagtgggtgtcaaacaagtggcttcatgagaggggacaagagtttagaaggccatgcactctttctgagcttgagtgatgagctc

SEQ ID NO: 15 - protein, 567 aa, synthetic construct
  REGION 1..567: note = Synthetic sequence containing the vacuolar signal sequence of barley gene for Thiol protease aleurain precursor fused to the human Prolyl 4-hydroxylase alpha-1 subunit and flanking regions
MAHARVLLLALAVLATAAVAVASSSSFADSNPIRPVTDRAASTLAQLVDMHPGFFTSIGQMTDLIHTEKDLVTSLKDYIKAEEDKLEQIKKWAEKLDRLTSTATKDPEGFVGHPVNAFKLMKRLNTEWSELENLVLKDMSDGFISNLTIQRQYFPNDEDQVGAAKALLRLQDTYNLDTDTISKGNLPGVKHKSFLTAEDCFELGKVAYTEADYYHTELWMEQALRQLDEGEISTIDKVSVLDYLSYAVYQQGDLDKALLLTKKLLELDPEHQRANGNLKYFEYIMAKEKDVNKSASDDQSDQKTTPKKKGVAVDYLPERQKYEMLCRGEGIKMTPRRQKKLFCRYHDGNRNPKFILAPAKQEDEWDKPRIIRFHDIISDAEIEIVKDLAKPRLRRATISNPITGDLETVHYRISKSAWLSGYENPVVSRINMRIQDLTGLDVSTAEELQVANYGVGGQYEPHFDFARKDEPDAFKELGTGNRIATWLFYMSDVSAGGATVFPEVGASVWPKKGTAVFWYNLFASGEGDYSTRHAACPVLVGNKWVSNKWLHERGQEFRRPCTLSELE

SEQ ID NO: 16 - DNA, 928 bp, synthetic construct
  misc_feature 1..928: note = Synthetic sequence containing the coding regions of the vacuolar signal sequence of barley gene for Thiol protease aleurain precursor fused to the plant Prolyl 4-hydroxylase Plant and flanking regions
  source 1..928: mol_type = other DNA
ctcgagtaaaccatggctcatgctagggttttgcttttggctcttgctgttcttgctactgctgctgttgctgtggcttcttcttcatctttcgctgattctaacccaattaggccagtgactgatagagctgcttctactcttgctcaattggtcgacatgcttggtattctttctcttccaaacgctaacaggaactcttctaagactaacgatcttactaacattgtgaggaagtctgagacttcttctggagatgaggagggaaatggagaaagatgggtggaagtgatttcttgggagccaagggctgttgtttaccacaacttccttactaatgaggagtgcgagcaccttatttctcttgctaagccatctatggtgaagtctactgtggtggatgagaaaactggaggatctaaggattcaagagtgaggacttcatctggtactttccttaggaggggacatgatgaagttgtggaagttattgagaagaggatttctgatttcactttcattccagtggagaacggagaaggacttcaagttcttcactaccaagtgggacaaaagtacgagccacactacgattacttccttgatgagttcaacactaagaacggaggacagaggattgctactgtgcttatgtacctttctgatgtggatgatggaggagagactgtttttccagctgctaggggaaacatttctgctgttccttggtggaacgagctttctaagtgtggaaaggagggactttctgtgcttccaaagaaaagggatgctcttcttttctggaacatgaggccagatgcttctcttgatccatcttctcttcatggaggatgcccagttgttaagggaaacaagtggtcatctactaagtggttccacgtgcacgagttcaaggtgtaatgagctc

SEQ ID NO: 17 - protein, 302 aa, synthetic construct
  REGION 1..302: note = Synthetic sequence containing the vacuolar signal sequence of barley gene for Thiol protease aleurain precursor fused to the plant Prolyl 4-hydroxylase Plant and flanking regions
MAHARVLLLALAVLATAAVAVASSSSFADSNPIRPVTDRAASTLAQLVDMLGILSLPNANRNSSKTNDLTNIVRKSETSSGDEEGNGERWVEVISWEPRAVVYHNFLTNEECEHLISLAKPSMVKSTVVDEKTGGSKDSRVRTSSGTFLRRGHDEVVEVIEKRISDFTFIPVENGEGLQVLHYQVGQKYEPHYDYFLDEFNTKNGGQRIATVLMYLSDVDDGGETVFPAARGNISAVPWWNELSKCGKEGLSVLPKKRDALLFWNMRPDASLDPSSLHGGCPVVKGNKWSSTKWFHVHEFKV

SEQ ID NO: 18 - DNA, 2689 bp, synthetic construct
  misc_feature 1..2689: note = Synthetic sequence containing the coding regions of the human Procollagen C-proteinase and flanking regions
  source 1..2689: mol_type = other DNA
agatctatcgatgcatgccatggtaccgcgccatggctcaattggctgcaacatcaaggcctgaaagagtttggccagatggtgttattcctttcgttattggtggaaactttactggatctcagagagcagtttttagacaagctatgagacattgggaaaagcacacttgtgtgacattccttgaaaggactgatgaagattcttatattgtgttcacataccgtccatgtggatgctgctcatatgttggtagaaggggaggaggtccacaagcaatttctattggaaaaaactgcgataagttcggaattgtggtgcatgaattgggacatgttgttggtttctggcacgaacacacaaggccagatagggataggcacgtgtctattgtgagggaaaacattcagccaggtcaagagtacaattttcttaagatggaacctcaagaggtggaatctctcggagagacttacgacttcgactccatcatgcactacgcaaggaatactttcagcaggggcatcttcttggataccattgtgcctaagtacgaggtgaacggcgttaagccacctattggtcaaaggactaggctctctaagggtgatattgcacaggctaggaagctctacaaatgtccagcatgcggagaaactcttcaggattccactggcaacttctcatctccagagtacccaaacggatactctgctcatatgcactgtgtttggaggatctcagtgactcctggagagaagatcatcctcaacttcacttccctcgatctctatcgttctaggctctgttggtacgactatgtggaagtgagagatggcttctggagaaaggctccacttagaggaaggttctgcggatctaaacttcctgagccaatcgtgtctactgattccagattgtgggtggagttcaggtcctcttctaattgggttggcaagggcttttttgctgtgtacgaggctatttgtggcggcgacgtgaaaaaggactacggacatattcaaagtccaaattacccagatgattaccgtccttcaaaagtgtgtatttggaggattcaagtgagtgagggtttccatgttggattgacattccaatctttcgaaattgagagacacgattcatgcgcatacgattatttggaagtgagagatggacactctgaatcttctacacttattggaaggtactgcggttatgagaaacctgatgatattaagtctacttctagtaggttgtggcttaaatttgtgtcagatggttctattaacaaggctggtttcgcagtgaacttcttcaaggaagtggatgaatgctcaagacctaacagaggaggatgtgagcaaagatgccttaacactttgggaagttacaagtgttcttgcgatcctggatacgagttggctcctgataagagaagatgcgaagctgcttgcggtggttttttgacaaaattgaacggatctattacttctcctggatggccaaaagagtacccacctaataagaattgcatttggcagcttgttgcacctactcagtaccgtatttcattgcaattcgattttttcgagactgagggtaatgatgtgtgcaagtacgatttcgtggaagtgagatcaggtcttactgctgatagtaaattgcacggaaagttctgcggatctgaaaaaccagaagtgattacatcacagtacaacaatatgagggtggagttcaaatctgataatactgtttctaaaaaaggttttaaggcacatttcttttctgataaggacgagtgctctaaagataatggtggttgccagcaggattgcgtgaacacattcggttcatatgagtgccaatgccgtagtggatttgttcttcacgataacaaacatgattgcaaagaggcaggttgcgatcacaaggtgacatctacttcaggtactatcacatctccaaactggcctgataagtatccttcaaaaaaagaatgtacatgggcaatttcttctacaccaggtcatagggttaagttgacattcatggagatggatattgagagtcaaccagagtgcgcttatgatcatcttgaggtgttcgatggaagggatgctaaggctcctgttcttggtagattctgtggtagtaaaaagccagaaccagtgcttgcaacaggatctaggatgttccttagattctactctgataactcagttcagaggaaaggattccaagctagtcacgcaactgaatgcggtggacaagttagagcagatgttaagactaaggatctttactcacacgcacagttcggagataacaactaccctggaggagttgattgcgagtgggttattgtggctgaagagggatacggagttgagcttgttttccagacattcgaggtggaggaggaaactgattgcggttacgattatatggaactttttgatggatacgatagtactgctccaagacttggaaggtattgtggtagtggtccaccagaagaggtgtactcagctggagatagtgttcttgttaagttccacagtgatgatacaattactaagaagggattccatcttagatatacttcaactaagtttcaggatactcttcattctaggaagtaatgagctcgcggccgcatccaagcttctgcagacgcgtcgacgtc

SEQ ID NO: 19 - protein, 870 aa, synthetic construct
  REGION 1..870: note = Synthetic sequence containing the human Procollagen C-proteinase and flanking regions
MAQLAATSRPERVWPDGVIPFVIGGNFTGSQRAVFRQAMRHWEKHTCVTFLERTDEDSYIVFTYRPCGCCSYVGRRGGGPQAISIGKNCDKFGIVVHELGHVVGFWHEHTRPDRDRHVSIVRENIQPGQEYNFLKMEPQEVESLGETYDFDSIMHYARNTFSRGIFLDTIVPKYEVNGVKPPIGQRTRLSKGDIAQARKLYKCPACGETLQDSTGNFSSPEYPNGYSAHMHCVWRISVTPGEKIILNFTSLDLYRSRLCWYDYVEVRDGFWRKAPLRGRFCGSKLPEPIVSTDSRLWVEFRSSSNWVGKGFFAVYEAICGGDVKKDYGHIQSPNYPDDYRPSKVCIWRIQVSEGFHVGLTFQSFEIERHDSCAYDYLEVRDGHSESSTLIGRYCGYEKPDDIKSTSSRLWLKFVSDGSINKAGFAVNFFKEVDECSRPNRGGCEQRCLNTLGSYKCSCDPGYELAPDKRRCEAACGGFLTKLNGSITSPGWPKEYPPNKNCIWQLVAPTQYRISLQFDFFETEGNDVCKYDFVEVRSGLTADSKLHGKFCGSEKPEVITSQYNNMRVEFKSDNTVSKKGFKAHFFSDKDECSKDNGGCQQDCVNTFGSYECQCRSGFVLHDNKHDCKEAGCDHKVTSTSGTITSPNWPDKYPSKKECTWAISSTPGHRVKLTFMEMDIESQPECAYDHLEVFDGRDAKAPVLGRFCGSKKPEPVLATGSRMFLRFYSDNSVQRKGFQASHATECGGQVRADVKTKDLYSHAQFGDNNYPGGVDCEWVIVAEEGYGVELVFQTFEVEEETDCGYDYMELFDGYDSTAPRLGRYCGSGPPEEVYSAGDSVLVKFHSDDTITKKGFHLRYTSTKFQDTLHSRK

SEQ ID NO: 20 - DNA, 2912 bp, synthetic construct
  misc_feature 1..2912: note = Synthetic sequence containing the coding regions of the human Procollagen I N-proteinase and flanking regions
  source 1..2912: mol_type = other DNA
gcgccatggctcaattgaggagaagggctaggagacacgcagctgatgatgattacaacattgaagttttgcttggtgttgatgatagtgtggtgcaattccacggaaaagagcatgttcagaaatatcttttgacacttatgaatattgtgaacgaaatctaccatgatgagtctttgggagcacacattaacgtggttcttgtgaggattattcttctttcatacggtaaatctatgtcacttattgagattggaaacccttctcagtctcttgagaatgtgtgcagatgggcataccttcaacagaagcctgatactggacacgatgagtatcacgatcacgctattttccttacaaggcaggatttcggtccaagtggaatgcaaggatatgctcctgttactggtatgtgccaccctgttaggtcttgtacacttaaccacgaggatggtttttcatctgctttcgtggtggctcatgagacaggtcatgttttgggaatggaacatgatggacagggtaatagatgtggagatgaagtgagacttggttcaattatggctcctcttgttcaagctgcttttcataggttccactggagtaggtgttcacagcaagagttgagtagataccttcattcttacgattgcttgcttgatgatccatttgctcatgattggccagctttgcctcaacttcctggattgcactactctatgaacgagcagtgcagatttgatttcggtcttggttacatgatgtgcacagctttcaggactttcgatccatgcaaacagttgtggtgttcacacccagataacccatatttctgtaaaacaaaaaaaggtccaccacttgatggtactatgtgcgcacctggaaagcactgcttcaagggacactgcatttggcttactcctgatattcttaaaagggatggatcatggggagcttggtctccattcggaagttgctcaagaacttgcggaacaggtgttaagtttagaactaggcagtgcgataatccacaccctgctaatggtggtagaacttgctctggacttgcttacgattttcagttgtgttctaggcaagattgccctgatagtcttgctgattttagagaagagcaatgtagacagtgggatctttactttgagcacggcgacgctcagcaccactggcttccacacgagcatagagatgcaaaagaaaggtgtcacctttattgcgagagtagagagactggagaggtggtgtcaatgaagagaatggtgcacgatggtacaaggtgttcttataaggatgcattctctttgtgtgtgaggggagattgcaggaaagtgggttgtgatggagtgattggatctagtaagcaagaagataagtgcggagtgtgcggaggagataactctcattgcaaggttgtgaaaggaacttttacaagatcaccaaaaaaacacggttacattaagatgttcgaaattcctgctggagcaaggcatttgcttattcaggaagtggatgcaacatctcaccacttggcagtgaaaaaccttgagactggaaaattcattttgaacgaggagaacgatgttgatgcatctagtaagactttcattgcaatgggtgttgaatgggagtatagggatgaggatggaagggaaacacttcaaacaatgggtcctcttcatggaacaattactgtgttggtgattccagtgggagatacaagggtgtcattgacatacaagtatatgattcacgaggatagtcttaacgttgatgataacaacgttttggaagaagattctgtggtttacgagtgggctcttaagaaatggtcaccttgctctaagccatgtggtggaggaagtcagttcactaagtatggttgtaggaggaggcttgatcataagatggttcataggggattttgcgcagcacttagtaagccaaaggcaattaggagggcttgtaaccctcaagaatgctcacaaccagtttgggtgacaggagagtgggagccatgttcacaaacatgcggaagaactggaatgcaagttagatcagttagatgcattcaacctcttcatgataacactacaagaagtgtgcacgcaaaacactgtaacgatgctaggccagagagtagaagagcttgctctagggaactttgccctggtagatggagggcaggaccttggagtcagtgctctgtgacatgtggaaacggtactcaggaaagacctgttccatgtagaactgctgatgatagtttcggaatttgtcaggaggaaaggccagaaacagctaggacttgtagacttggaccttgtcctaggaatatttctgatcctagtaaaaaatcatacgtggtgcaatggttgagtaggccagatccagattcaccaattaggaagatttcttcaaaaggacactgccagggtgataagagtattttctgcagaatggaagttcttagtaggtactgttctattccaggttataacaaactttcttgtaagagttgcaacttgtataacaatcttactaacgtggagggtagaattgaacctccaccaggaaagcacaacgatattgatgtgtttatgcctactcttcctgtgccaacagttgcaatggaagttagaccttctccatctactccacttgaggtgccacttaatgcatcaagtactaacgctactgaggatcacccagagactaacgcagttgatgagccttataagattcacggacttgaggatgaggttcagccaccaaaccttattcctaggaggccaagtccttacgaaaaaactagaaatcagaggattcaggagcttattgatgagatgaggaaaaaggagatgcttggaaagttctaatgagctcgcggccgcatc

SEQ ID NO: 21 - protein, 962 aa, synthetic construct
  REGION 1..962: note = Synthetic sequence containing the human Procollagen I N-proteinase and flanking regions
MAQLRRRARRHAADDDYNIEVLLGVDDSVVQFHGKEHVQKYLLTLMNIVNEIYHDESLGAHINVVLVRIILLSYGKSMSLIEIGNPSQSLENVCRWAYLQQKPDTGHDEYHDHAIFLTRQDFGPSGMQGYAPVTGMCHPVRSCTLNHEDGFSSAFVVAHETGHVLGMEHDGQGNRCGDEVRLGSIMAPLVQAAFHRFHWSRCSQQELSRYLHSYDCLLDDPFAHDWPALPQLPGLHYSMNEQCRFDFGLGYMMCTAFRTFDPCKQLWCSHPDNPYFCKTKKGPPLDGTMCAPGKHCFKGHCIWLTPDILKRDGSWGAWSPFGSCSRTCGTGVKFRTRQCDNPHPANGGRTCSGLAYDFQLCSRQDCPDSLADFREEQCRQWDLYFEHGDAQHHWLPHEHRDAKERCHLYCESRETGEVVSMKRMVHDGTRCSYKDAFSLCVRGDCRKVGCDGVIGSSKQEDKCGVCGGDNSHCKVVKGTFTRSPKKHGYIKMFEIPAGARHLLIQEVDATSHHLAVKNLETGKFILNEENDVDASSKTFIAMGVEWEYRDEDGRETLQTMGPLHGTITVLVIPVGDTRVSLTYKYMIHEDSLNVDDNNVLEEDSVVYEWALKKWSPCSKPCGGGSQFTKYGCRRRLDHKMVHRGFCAALSKPKAIRRACNPQECSQPVWVTGEWEPCSQTCGRTGMQVRSVRCIQPLHDNTTRSVHAKHCNDARPESRRACSRELCPGRWRAGPWSQCSVTCGNGTQERPVPCRTADDSFGICQEERPETARTCRLGPCPRNISDPSKKSYVVQWLSRPDPDSPIRKISSKGHCQGDKSIFCRMEVLSRYCSIPGYNKLSCKSCNLYNNLTNVEGRIEPPPGKHNDIDVFMPTLPVPTVAMEVRPSPSTPLEVPLNASSTNATEDHPETNAVDEPYKIHGLEDEVQPPNLIPRRPSPYEKTRNQRIQELIDEMRKKEMLGKF

SEQ ID NO: 22 - DNA, 2888 bp, synthetic construct
  misc_feature 1..2888: note = Synthetic sequence containing the coding regions of the vacuolar signal sequence of barley gene for Thiol protease aleurain precursor fused to the human Lysyl hydroxylase 3 and flanking regions
  source 1..2888: mol_type = other DNA
gcgaattcgctagctatcactgaaaagacagcaagacaatggtgtctcgatgcaccagaaccacatctttgcagcagatgtgaagcagccagagtggtccacaagacgcactcagaaaaggcatcttctaccgacacagaaaaagacaaccacagctcatcatccaacatgtagactgtcgttatgcgtcggctgaagataagactgaccccaggccagcactaaagaagaaataatgcaagtggtcctagctccactttagctttaataattatgtttcattattattctctgcttttgctctctatataaagagcttgtattttcatttgaaggcagaggcgaacacacacacagaacctccctgcttacaaaccagatcttaaaccatggctcacgctagggttttgcttcttgctcttgctgttcttgctactgctgctgttgctgtggcttcttcaagttctttcgctgattctaacccaattaggccagtgactgatagagctgcttctactcttgctcaattgagatctatgtctgatagaccaaggggaagggatccagttaatccagagaagttgcttgtgattactgtggctactgctgagactgaaggataccttagattccttaggagtgctgagttcttcaactacactgtgaggactcttggacttggagaagaatggaggggaggagatgttgctagaactgttggaggaggacagaaagtgagatggcttaagaaagagatggagaagtacgctgatagggaggatatgattattatgttcgtggattcttacgatgtgattcttgctggatctccaactgagcttttgaagaaattcgttcagtctggatctaggcttcttttctctgctgagtctttttgttggccagaatggggacttgctgagcaatatccagaagtgggaactggaaagagattccttaactctggaggattcattggattcgctactactattcaccagattgtgaggcagtggaagtacaaggatgacgatgatgatcagcttttctacactaggctttaccttgatccaggacttagggagaagttgtctcttaaccttgatcacaagtctaggattttccagaaccttaacggtgctcttgatgaggttgtgcttaagttcgataggaacagagtgaggattaggaacgtggcttacgatactcttcctattgtggtgcatggaaacggaccaacaaaactccagcttaactaccttggaaactacgttccaaacggatggactccagaaggaggatgtggattctgcaatcaggataggagaactcttccaggaggacaaccaccaccaagagttttccttgctgtgttcgttgaacagccaactccattccttccaagattccttcagaggcttcttcttttggattacccaccagatagggtgacacttttccttcacaacaacgaggttttccacgagccacacattgctgattcttggccacagcttcaggatcatttctctgctgtgaagttggttggtccagaagaagctctttctccaggagaagctagggatatggctatggatttgtgcaggcaggatccagagtgcgagttctacttctctcttgatgctgatgctgtgcttactaaccttcagactcttaggattcttattgaggagaacaggaaagtgattgctccaatgctttctaggcacggaaagttgtggtctaatttctggggtgctctttctcctgatgagtactacgctagatcagaggactacgtggagcttgttcagagaaagagagtgggagtttggaacgttccttatatttctcaggcttacgtgattaggggagatactcttaggatggagcttccacagagggatgttttctctggatctgatactgatccagatatggctttctgcaagtctttcagggataagggaattttccttcacctttctaaccagcatgagttcggaagattgcttgctacttcaagatacgatactgagcaccttcatcctgatctttggcagattttcgataacccagtggattggaaggagcagtacattcacgagaactactctagggctcttgaaggagaaggaattgtggagcaaccatgcccagatgtttactggttcccacttctttctgagcaaatgtgcgatgagcttgttgctgagatggagcattacggacaatggagtggaggtagacatgaggattctaggcttgctggaggatacgagaacgttccaactgtggatattcacatgaagcaagtgggatacgaggatcaatggcttcagcttcttaggacttatgtgggaccaatgactgagtctcttttcccaggataccacactaaggctagggctgttatgaacttcgttgtgaggtatcgtccagatgagcaaccatctcttaggccacaccacgattcttctactttcactcttaacgtggctcttaaccacaagggacttgattatgagggaggaggatgccgtttccttagatacgattgcgtgatttcttcaccaagaaagggatgggctcttcttcatccaggaaggcttactcattaccacgagggacttccaactacttggggaactagatatattatggtgtctttcgtggatccatgactgctttaatgagatatgcgagacgcctatgatcgcatgatatttgctttcaattctgttgtgcacgttgtaaaaaacctgagcatgtgtagctcagatccttaccgccggtttcggttcattctaatgaatatatcacccgttactatcgtatttttatgaataatattctccgttcaatttactgattgtccagaattcgcg

SEQ ID NO: 23 - protein, 764 aa, synthetic construct
  REGION 1..764: note = Synthetic sequence containing the vacuolar signal sequence of barley gene for Thiol protease aleurain precursor fused to the human Lysyl hydroxylase 3 and flanking regions
MAHARVLLLALAVLATAAVAVASSSSFADSNPIRPVTDRAASTLAQLRSMSDRPRGRDPVNPEKLLVITVATAETEGYLRFLRSAEFFNYTVRTLGLGEEWRGGDVARTVGGGQKVRWLKKEMEKYADREDMIIMFVDSYDVILAGSPTELLKKFVQSGSRLLFSAESFCWPEWGLAEQYPEVGTGKRFLNSGGFIGFATTIHQIVRQWKYKDDDDDQLFYTRLYLDPGLREKLSLNLDHKSRIFQNLNGALDEVVLKFDRNRVRIRNVAYDTLPIVVHGNGPTKLQLNYLGNYVPNGWTPEGGCGFCNQDRRTLPGGQPPPRVFLAVFVEQPTPFLPRFLQRLLLLDYPPDRVTLFLHNNEVFHEPHIADSWPQLQDHFSAVKLVGPEEALSPGEARDMAMDLCRQDPECEFYFSLDADAVLTNLQTLRILIEENRKVIAPMLSRHGKLWSNFWGALSPDEYYARSEDYVELVQRKRVGVWNVPYISQAYVIRGDTLRMELPQRDVFSGSDTDPDMAFCKSFRDKGIFLHLSNQHEFGRLLATSRYDTEHLHPDLWQIFDNPVDWKEQYIHENYSRALEGEGIVEQPCPDVYWFPLLSEQMCDELVAEMEHYGQWSGGRHEDSRLAGGYENVPTVDIHMKQVGYEDQWLQLLRTYVGPMTESLFPGYHTKARAVMNFVVRYRPDEQPSLRPHHDSSTFTLNVALNHKGLDYEGGGCRFLRYDCVISSPRKGWALLHPGRLTHYHEGLPTTWGTRYIMVSFVDP

SEQ ID NO: 24 - protein, 45 aa, synthetic construct
  REGION 1..45: note = Vacuole signal sequence of barley gene for Thiol protease aleurain precursor
MAHARVLLLALAVLATAAVAVASSSSFADSNPIRPVTDRAASTLA

SEQ ID NO: 25 - DNA, 24 bp, synthetic construct
  misc_feature 1..24: note = Single strand DNA oligonucleotide
  source 1..24: mol_type = other DNA
atcaccaggagaacagggaccatc

SEQ ID NO: 26 - DNA, 29 bp, synthetic construct
  misc_feature 1..29: note = Single strand DNA oligonucleotide
  source 1..29: mol_type = other DNA
tccacttccaaatctctatccctaacaac

SEQ ID NO: 27 - DNA, 23 bp, synthetic construct
  misc_feature 1..23: note = Single strand DNA oligonucleotide
  source 1..23: mol_type = other DNA
aggcattagaggcgataagggag

SEQ ID NO: 28 - DNA, 27 bp, synthetic construct
  misc_feature 1..27: note = Single strand DNA oligonucleotide
  source 1..27: mol_type = other DNA
tcaatccaataatagccacttgaccac

SEQ ID NO: 29 - DNA, 102 bp, synthetic construct
  misc_feature 1..102: note = pBINPLUS multiple cloning site
  source 1..102: mol_type = other DNA
atgaccatgattacgccaagctggcgcgccaagcttgcatgcctgcaggtcgactctagaggatccccgggtaccgagctcgaattcttaattaacaattca

SEQ ID NO: 30 - protein, 1464 aa, Homo sapiens
MFSFVDLRLLLLLAATALLTHGQEEGQVEGQDEDIPPITCVQNGLRYHDRDVWKPEPCRICVCDNGKVLCDDVICDETKNCPGAEVPEGECCPVCPDGSESPTDQETTGVEGPKGDTGPRGPRGPAGPPGRDGIPGQPGLPGPPGPPGPPGPPGLGGNFAPQLSYGYDEKSTGGISVPGPMGPSGPRGLPGPPGAPGPQGFQGPPGEPGEPGASGPMGPRGPPGPPGKNGDDGEAGKPGRPGERGPPGPQGARGLPGTAGLPGMKGHRGFSGLDGAKGDAGPAGPKGEPGSPGENGAPGQMGPRGLPGERGRPGAPGPAGARGNDGATGAAGPPGPTGPAGPPGFPGAVGAKGEAGPQGPRGSEGPQGVRGEPGPPGPAGAAGPAGNPGADGQPGAKGANGAPGIAGAPGFPGARGPSGPQGPGGPPGPKGNSGEPGAPGSKGDTGAKGEPGPVGVQGPPGPAGEEGKRGARGEPGPTGLPGPPGERGGPGSRGFPGADGVAGPKGPAGERGSPGPAGPKGSPGEAGRPGEAGLPGAKGLTGSPGSPGPDGKTGPPGPAGQDGRPGPPGPPGARGQAGVMGFPGPKGAAGEPGKAGERGVPGPPGAVGPAGKDGEAGAQGPPGPAGPAGERGEQGPAGSPGFQGLPGPAGPPGEAGKPGEQGVPGDLGAPGPSGARGERGFPGERGVQGPPGPAGPRGANGAPGNDGAKGDAGAPGAPGSQGAPGLQGMPGERGAAGLPGPKGDRGDAGPKGADGSPGKDGVRGLTGPIGPPGPAGAPGDKGESGPSGPAGPTGARGAPGDRGEPGPPGPAGFAGPPGADGQPGAKGEPGDAGAKGDAGPPGPAGPAGPPGPIGNVGAPGAKGARGSAGPPGATGFPGAAGRVGPPGPSGNAGPPGPPGPAGKEGGKGPRGETGPAGRPGEVGPPGPPGPAGEKGSPGADGPAGAPGTPGPQGIAGQRGVVGLPGQRGERGFPGLPGPSGEPGKQGPSGASGERGPPGPMGPPGLAGPPGESGREGAPGAEGSPGRDGSPGAKGDRGETGPAGPPGAPGAPGAPGPVGPAGKSGDRGETGPAGPAGPVGPVGARGPAGPQGPRGDKGETGEQGDRGIKGHRGFSGLQGPPGPPGSPGEQGPSGASGPAGPRGPPGSAGAPGKDGLNGLPGPIGPPGPRGRTGDAGPVGPPGPPGPPGPPGPPSAGFDFSFLPQPPQEKAHDGGRYYRADDANVVRDRDLEVDTTLKSLSQQIENIRSPEGSRKNPARTCRDLKMCHSDWKSGEYWIDPNQGCNLDAIKVFCNMETGETCVYPTQPSVAQKNWYISKNPKDKRHVWFGESMTDGFQFEYGGQGSDPADVAIQLTFLRLMSTEASQNITYHCKNSVAYMDQQTGNLKKALLLQGSNEIEIRAEGNSRFTYSVTVDGCTSHTGAWGKTVIEYKTTKTSRLPIIDVAPLDVGAPDQEFGFDVGPVCFL

SEQ ID NO: 31 - protein, 1366 aa, Homo sapiens [sequence omitted]

SEQ ID NO: 32 - DNA, 5927 bp, Homo sapiens
  source 1..5927: mol_type = genomic DNA
tcgtcggagcagacgggagtttctcctcggggtcggagcaggaggcacgcggagtgtgaggccacgcatgagcggacgctaaccccctccccagccacaaagagtctacatgtctagggtctagacatgttcagctttgtggacctccggctcctgctcctcttagcggccaccgccctcctgacgcacggccaagaggaaggccaagtcgagggccaagacgaagacatcccaccaatcacctgcgtacagaacggcctcaggtaccatgaccgagacgtgtggaaacccgagccctgccggatctgcgtctgcgacaacggcaaggtgttgtgcgatgacgtgatctgtgacgagaccaagaactgccccggcgccgaagtccccgagggcgagtgctgtcccgtctgccccgacggctcagagtcacccaccgaccaagaaaccaccggcgtcgagggacccaagggagacactggcccccgaggcccaaggggacccgcaggcccccctggccgagatggcatccctggacagcctggacttcccggaccccccggaccccccggacctcccggaccccctggcctcggaggaaactttgctccccagctgtcttatggctatgatgagaaatcaaccggaggaatttccgtgcctggccccatgggtccctctggtcctcgtggtctccctggcccccctggtgcacctggtccccaaggcttccaaggtccccctggtgagcctggcgagcctggagcttcaggtcccatgggtccccgaggtcccccaggtccccctggaaagaatggagatgatggggaagctggaaaacctggtcgtcctggtgagcgtgggcctcctgggcctcagggtgctcgaggattgcccggaacagctggcctccctggaatgaagggacacagaggtttcagtggtttggatggtgccaagggagatgctggtcctgctggtcctaagggtgagcctggcagccctggtgaaaatggagctcctggtcagatgggcccccgtggcctgcctggtgagagaggtcgccctggagcccctggccctgctggtgctcgtggaaatgatggtgctactggtgctgccgggccccctggtcccaccggccccgctggtcctcctggcttccctggtgctgttggtgctaagggtgaagctggtccccaagggccccgaggctctgaaggtccccagggtgtgcgtggtgagcctggcccccctggccctgctggtgctgctggccctgctggaaaccctggtgctgatggacagcctggtgctaaaggtgccaatggtgctcctggtattgctggtgctcctggcttccctggtgcccgaggcccctctggaccccagggccccggcggccctcctggtcccaagggtaacagcggtgaacctggtgctcctggcagcaaaggagacactggtgctaagggagagcctggccctgttggtgttcaaggaccccctggccctgctggagaggaaggaaagcgaggagctcgaggtgaacccggacccactggcctgcccggaccccctggcgagcgtggtggacctggtagccgtggtttccctggcgcagatggtgttgctggtcccaagggtcccgctggtgaacgtggttctcctggccctgctggccccaaaggatctcctggtgaagctggtcgtcccggtgaagctggtctgcctggtgccaagggtctgactggaagccctggcagccctggtcctgatggcaaaactggcccccctggtcccgccggtcaagatggtcgccccggacccccaggcccacctggtgcccgtggtcaggctggtgtgatgggattccctggacctaaaggtgctgctggagagcccggcaaggctggagagcgaggtgttcccggaccccctggcgctgtcggtcctgctggcaaagatggagaggctggagctcagggaccccctggccctgctggtcccgctggcgagagaggtgaacaaggccctgctggctcccccggattccagggtctccctggtcctgctggtcctccaggtgaagcaggcaaacctggtgaacagggtgttcctggagaccttggcgcccctggcccctctggagcaagaggcgagagaggtttccctggcgagcgtggtgtgcaaggtccccctggtcctgctggtccccgaggggccaacggtgctcccggcaacgatggtgctaagggtgatgctggtgcccctggagctcccggtagccagggcgcccctggccttcagggaatgcctggtgaacgtggtgcagctggtcttccagggcctaagggtgacagaggtgatgctggtcccaaaggtgctgatggctctcctggcaaagatggcgtccgtggtctgactggccccattggtcctcctggccctgctggtgcccctggtgacaagggtgaaagtggtcccagcggccctgctggtcccactggagctcgtggtgcccccggagaccgtggtgagcctggtccccccggccctgctggctttgctggcccccctggtgctgacggccaacctggtgctaaaggcgaacctggtgatgctggtgctaaaggcgatgctggtccccctggccctgccggacccgctggaccccctggccccattggtaatgttggtgctcctggagccaaaggtgctcgcggcagcgctggtccccctggtgctactggtttccctggtgctgctggccgagtcggtcctcctggcccctctggaaatgctggaccccctggccctcctggtcctgctggcaaagaaggcggcaaaggtccccgtggtgagactggccctgctggacgtcctggtgaagttggtccccctggtccccctggccctgctggcgagaaaggatcccctggtgctgatggtcctgctggtgctcctggtactcccgggcctcaaggtattgctggacagcgtggtgtggtcggcctgcctggtcagagaggagagagaggcttccctggtcttcctggcccctctggtgaacctggcaaacaaggtccctctggagcaagtggtgaacgtggtccccctggtcccatgggcccccctggattggctggaccccctggtgaatctggacgtgagggggctcctggtgccgaaggttcccctggacgagacggttctcctggcgccaagggtgaccgtggtgagaccggccccgctggaccccctggtgctcctggtgctcctggtgcccctggccccgttggccctgctggcaagagtggtgatcgtggtgagactggtcctgctggtcccgccggtcctgtcggccctgttggcgcccgtggccccgccggaccccaaggcccccgtggtgacaagggtgagacaggcgaacagggcgacagaggcataaagggtcaccgtggcttctctggcctccagggtccccctggccctcctggctctcctggtgaacaaggtccctctggagcctctggtcctgctggtccccgaggtccccctggctctgctggtgctcctggcaaagatggactcaacggtctccctggccccattgggccccctggtcctcgcggtcgcactggtgatgctggtcctgttggtccccccggccctcctggacctcctggtccccctggtcctcccagcgctggtttcgacttcagcttcctgccccagccacctcaagagaaggctcacgatggtggccgctactaccgggctgatgatgccaatgtggttcgtgaccgtgacctcgaggtggacaccaccctcaagagcctgagccagcagatcgagaacatccggagcccagagggcagccgcaagaaccccgcccgcacctgccgtgacctcaagatgtgccactctgactggaagagtggagagtactggattgaccccaaccaaggctgcaacctggatgccatcaaagtcttctgcaacatggagactggtgagacctgcgtgtaccccactcagcccagtgtggcccagaagaactggtacatcagcaagaaccccaaggacaagaggcatgtctggttcggcgagagcatgaccgatggattccagttcgagtatggcggccagggctccgaccctgccgatgtggccatccagctgaccttcctgcgcctgatgtccaccgaggcctcccagaacatcacctaccactgcaagaacagcgtggcctacatggaccagcagactggcaacctcaagaaggccctgctcctccagggctccaacgagatcgagatccgcgccgagggcaacagccgcttcacctacagcgtcactgtcgatggctgcacgagtcacaccggagcctggggcaagacagtgattgaatacaaaaccaccaagacctcccgcctgcccatcatcgatgtggcccccttggacgttggtgccccagaccaggaattcggcttcgacgttggccctgtctgcttcctgtaaactccctccatcccaacctggctccctcccacccaaccaactttccccccaacccggaaacagacaagcaacccaaactgaaccccctcaaaagccaaaaaatgggagacaatttcacatggactttggaaaatatttttttcctttgcattcatctctcaaacttagtttttatctttgaccaaccgaacatgaccaaaaaccaaaagtgcattcaaccttaccaaaaaaaaaaaaaaaaaaagaataaataaataactttttaaaaaaggaagcttggtccacttgcttgaagacccatgcgggggtaagtccctttctgcccgttgggcttatgaaaccccaatgctgccctttctgctcctttctccacaccccccttggggcctcccctccactccttcccaaatctgtctccccagaagacacaggaaacaatgtattgtctgcccagcaatcaaaggcaatgctcaaacacccaagtggcccccaccctcagcccgctcctgcccgcccagcacccccaggccctgggggacctggggttctcagactgccaaagaagccttgccatctggcgctcccatggctcttgcaacatctccccttcgtttttgagggggtcatgccgggggagccaccagcccctcactgggttcggaggagagtcaggaagggccacgacaaagcagaaacatcggatttggggaacgcgtgtcaatcccttgtgccgcagggctgggcgggagagactgttctgttccttgtgtaactgtgttgctgaaagactacctcgttcttgtcttgatgtgtcaccggggcaactgcctgggggcggggatgggggcagggtggaagcggctccccattttataccaaaggtgctacatctatgtgatgggtggggtggggagggaatcactggtgctatagaaattgagatgcccccccaggccagcaaatgttcctttttgttcaaagtctatttttattccttgatatttttctttttttttttttttttttgtggatggggacttgtgaatttttctaaaggtgctatttaacatgggaggagagcgtgtgcggctccagcccagcccgctgctcactttccaccctctctccacctgcctctggcttctcaggcctctgctctccgacctctctcctctgaaaccctcctccacagctgcagcccatcctcccggctccctcctagtctgtcctgcgtcctctgtccccgggtttcagagacaacttcccaaagcacaaagcagtttttccccctaggggtgggaggaagcaaaagactctgtacctattttgtatgtgtataataatttgagatgtttttaattattttgattgctggaataaagcatgtggaaatgacccaaacataa

SEQ ID NO: 33 - DNA, 5411 bp, Homo sapiens
  source 1..5411: mol_type = genomic DNA
gtgtcccatagtgtttccaaacttggaaagggcgggggagggcgggaggatgcggagggcggaggtatgcagacaacgagtcagagtttccccttgaaagcctcaaaagtgtccacgtcctcaaaaagaatggaaccaatttaagaagccagccccgtggccacgtcccttcccccattcgctccctcctctgcgcccccgcaggctcctcccagctgtggctgcccgggcccccagccccagccctcccattggtggaggcccttttggaggcaccctagggccagggaaacttttgccgtataaatagggcagatccgggctttattattttagcaccacggcagcaggaggtttcggctaagttggaggtactggccacgactgcatgcccgcgcccgccaggtgatacctccgccggtgacccaggggctctgcgacacaaggagtctgcatgtctaagtgctagacatgctcagctttgtggatacgcggactttgttgctgcttgcagtaaccttatgcctagcaacatgccaatctttacaagaggaaactgtaagaaagggcccagccggagatagaggaccacgtggagaaaggggtccaccaggccccccaggcagagatggtgaagatggtcccacaggccctcctggtccacctggtcctcctggcccccctggtctcggtgggaactttgctgctcagtatgatggaaaaggagttggacttggccctggaccaatgggcttaatgggacctagaggcccacctggtgcagctggagccccaggccctcaaggtttccaaggacctgctggtgagcctggtgaacctggtcaaactggtcctgcaggtgctcgtggtccagctggccctcctggcaaggctggtgaagatggtcaccctggaaaacccggacgacctggtgagagaggagttgttggaccacagggtgctcgtggtttccctggaactcctggacttcctggcttcaaaggcattaggggacacaatggtctggatggattgaagggacagcccggtgctcctggtgtgaagggtgaacctggtgcccctggtgaaaatggaactccaggtcaaacaggagcccgtgggcttcctggtgagagaggacgtgttggtgcccctggcccagctggtgcccgtggcagtgatggaagtgtgggtcccgtgggtcctgctggtcccattgggtctgctggccctccaggcttcccaggtgcccctggccccaagggtgaaattggagctgttggtaacgctggtcctgctggtcccgccggtccccgtggtgaagtgggtcttccaggcctctccggccccgttggacctcctggtaatcctggagcaaacggccttactggtgccaagggtgctgctggccttcccggcgttgctggggctcccggcctccctggaccccgcggtattcctggccctgttggtgctgccggtgctactggtgccagaggacttgttggtgagcctggtccagctggctccaaaggagagagcggtaacaagggtgagcccggctctgctgggccccaaggtcctcctggtcccagtggtgaagaaggaaagagaggccctaatggggaagctggatctgccggccctccaggacctcctgggctgagaggtagtcctggttctcgtggtcttcctggagctgatggcagagctggcgtcatgggccctcctggtagtcgtggtgcaagtggccctgctggagtccgaggacctaatggagatgctggtcgccctggggagcctggtctcatgggacccagaggtcttcctggttcccctggaaatatcggccccgctggaaaagaaggtcctgtcggcctccctggcatcgacggcaggcctggcccaattggcccagctggagcaagaggagagcctggcaacattggattccctggacccaaaggccccactggtgatcctggcaaaaacggtgataaaggtcatgctggtcttgctggtgctcggggtgctccaggtcctgatggaaacaatggtgctcagggacctcctggaccacagggtgttcaaggtggaaaaggtgaacagggtccccctggtcctccaggcttccagggtctgcctggcccctcaggtcccgctggtgaagttggcaaaccaggagaaaggggtctccatggtgagtttggtctccctggtcctgctggtccaagaggggaacgcggtcccccaggtgagagtggtgctgccggtcctactggtcctattggaagccgaggtccttctggacccccagggcctgatggaaacaagggtgaacctggtgtggttggtgctgtgggcactgctggtccatctggtcctagtggactcccaggagagaggggtgctgctggcatacctggaggcaagggagaaaagggtgaacctggtctcagaggtgaaattggtaaccctggcagagatggtgctcgtggtgctcctggtgctgtaggtgcccctggtcctgctggagccacaggtgaccggggcgaagctggggctgctggtcctgctggtcctgctggtcctcggggaagccctggtgaacgtggtgaggtcggtcctgctggccccaatggatttgctggtcctgctggtgctgctggtcaacctggtgctaaaggagaaagaggagccaaagggcctaagggtgaaaacggtgttgttggtcccacaggccccgttggagctgctggcccagctggtccaaatggtccccccggtcctgctggaagtcgtggtgatggaggcccccctggtatgactggtttccctggtgctgctggacggactggtcccccaggaccctctggtatttctggccctcctggtccccctggtcctgctgggaaagaagggcttcgtggtcctcgtggtgaccaaggtccagttggccgaactggagaagtaggtgcagttggtccccctggcttcgctggtgagaagggtccctctggagaggctggtactgctggacctcctggcactccaggtcctcagggtcttcttggtgctcctggtattctgggtctccctggctcgagaggtgaacgtggtctaccaggtgttgctggtgctgtgggtgaacctggtcctcttggcattgccggccctcctggggcccgtggtcctcctggtgctgtgggtagtcctggagtcaacggtgctcctggtgaagctggtcgtgatggcaaccctgggaacgatggtcccccaggtcgcgatggtcaacccggacacaagggagagcgcggttaccctggcaatattggtcccgttggtgctgcaggtgcacctggtcctcatggccccgtgggtcctgctggcaaacatggaaaccgtggtgaaactggtccttctggtcctgttggtcctgctggtgctgttggcccaagaggtcctagtggcccacaaggcattcgtggcgataagggagagcccggtgaaaaggggcccagaggtcttcctggcttaaagggacacaatggattgcaaggtctgcctggtatcgctggtcaccatggtgatcaaggtgctcctggctccgtgggtcctgctggtcctaggggccctgctggtccttctggccctgctggaaaagatggtcgcactggacatcctggtacagttggacctgctggcattcgaggccctcagggtcaccaaggccctgctggcccccctggtccccctggccctcctggacctccaggtgtaagcggtggtggttatgactttggttacgatggagacttctacagggctgaccagcctcgctcagcaccttctctcagacccaaggactatgaagttgatgctactctgaagtctctcaacaaccagattgagacccttcttactcctgaaggctctagaaagaacccagctcgcacatgccgtgacttgagactcagccacccagagtggagcagtggttactactggattgaccctaaccaaggatgcactatggatgctatcaaagtatactgtgatttctctactggcgaaacctgtatccgggcccaacctgaaaacatcccagccaagaactggtataggagctccaaggacaagaaacacgtctggctaggagaaactatcaatgctggcagccagtttgaatataatgtagaaggagtgacttccaaggaaatggctacccaacttgccttcatgcgcctgctggccaactatgcctctcagaacatcacctaccactgcaagaacagcattgcatacatggatgaggagactggcaacctgaaaaaggctgtcattctacagggctctaatgatgttgaacttgttgctgagggcaacagcaggttcacttacactgttcttgtagatggctgctctaaaaagacaaatgaatggggaaagacaatcattgaatacaaaacaaataagccatcacgcctgcccttccttgatattgcacctttggacatcggtggtgctgaccaggaattctttgtggacattggcccagtctgtttcaaataaatgaactcaatctaaattaaaaaagaaagaaatttgaaaaaactttctctttgccatttcttcttcttcttttttaactgaaagctgaatccttccatttcttctgcacatctacttgcttaaattgtgggcaaaagagaaaaagaaggattgatcagagcattgtgcaatacagtttcattaactccttcccccgctcccccaaaaatttgaatttttttttcaacactcttacacctgttatggaaaatgtcaacctttgtaagaaaaccaaaataaaaattgaaaaataaaaaccataaacatttgcaccacttgtggcttttgaatatcttccacagagggaagtttaaaacccaaacttccaaaggtttaaactacctcaaaacactttcccatgagtgtgatccacattgttaggtgctgacctagacagagatgaactgaggtccttgttttgttttgttcataatacaaaggtgctaattaatagtatttcagatacttgaagaatgttgatggtgctagaagaatttgagaagaaatactcctgtattgagttgtatcgtgtggtgtattttttaaaaaatttgatttagcattcatattttccatcttattcccaattaaaagtatgcagattatttgcccaaatcttcttcagattcagcatttgttctttgccagtctcattttcatcttcttccatggttccacagaagctttgtttcttgggcaagcagaaaaattaaattgtacctattttgtatatgtgagatgtttaaataaattgtgaaaaaaatgaaataaagcatgtttggttttccaaaagaacatat

SEQ ID NO: 34 - DNA, 1633 bp, synthetic construct; identical to SEQ ID NO: 12
  misc_feature 1..1633: note = Synthetic sequence containing the coding regions of the vascular signal sequence of barley gene for Thiol protease aleurain precursor fused to the human Prolyl 4-hydroxylase beta subunit and flanking regions
  source 1..1633: mol_type = other DNA

SEQ ID NO: 35 - DNA, 1723 bp, synthetic construct; identical to SEQ ID NO: 14
  misc_feature 1..1723: note = Synthetic sequence containing the coding regions of the vascular signal sequence of barley gene for Thiol protease aleurain precursor fused to the human Prolyl 4-hydroxylase alpha-1 subunit and flanking regions
  source 1..1723: mol_type = other DNA

SEQ ID NO: 36 - protein, 1489 aa, Homo sapiens; identical to SEQ ID NO: 3

SEQ ID NO: 37 - protein, 1389 aa, Homo sapiens; identical to SEQ ID NO: 6

SEQ ID NO: 38 - DNA, 2888 bp, synthetic construct; identical to SEQ ID NO: 22
  misc_feature 1..2888: note = Synthetic sequence containing the coding regions of the vascular signal sequence of barley gene for Thiol protease aleurain precursor fused to the human Lysyl hydroxylase 3 and flanking regions
  source 1..2888: mol_type = other DNA

SEQ ID NO: 39 - DNA, 2689 bp, synthetic construct; identical to SEQ ID NO: 18
  misc_feature 1..2689: note = Synthetic sequence containing the coding regions of the human Procollagen C-proteinase and flanking regions
  source 1..2689: mol_type = other DNA

SEQ ID NO: 40 - DNA, 2912 bp, synthetic construct; identical to SEQ ID NO: 20
  misc_feature 1..2912: note = Synthetic sequence containing the coding regions of the human Procollagen I N-proteinase and flanking regions
  source 1..2912: mol_type = other DNA

SEQ ID NO: 41 - DNA, 4467 bp, Homo sapiens
  source 1..4467: mol_type = genomic DNA
atggctcacgctcgtgttctcctcctcgctctcgctgttttggcaacagctgctgtggctgtggcttctagttcttcttttgctgattcaaaccctattagacctgttactgatagagcagcttccactttggctcaattgcaagaggagggccaggttgagggccaagatgaggatatccctccaattacatgcgtgcaaaatggcttgcgttaccacgatagggatgtgtggaaacctgaaccttgtcgtatctgtgtgtgtgataacggcaaggtgctctgcgatgatgttatctgcgatgagacaaaaaattgccctggcgctgaagttcctgagggcgagtgttgccctgtgtgccctgatggttccgagtccccaactgatcaggaaactactggcgtggagggcccaaaaggagatactggtccacgtggtcctaggggtccagcaggtcctccaggtagagatggtattccaggccagcctggattgccaggaccaccaggcccacctggcccaccaggacctcctggtcttggtggaaatttcgctccacaactctcttatggctatgatgagaagtcaacaggtggtatttccgttccaggtcctatgggaccatccggaccaagaggtctcccaggtcctccaggtgctcctggacctcaaggctttcaaggacctccaggcgaaccaggagaaccaggcgcttctggaccaatgggcccaaggggaccacctggcccaccaggaaaaaatggcgatgatggcgaagctggaaagcctggtcgtcctggagagagaggtcctcctggcccacagggtgcaagaggcttgccaggaactgctggcttgcctggaatgaagggacataggggcttctccggcctcgatggcgctaagggtgatgctggccctgctggaccaaagggcgagccaggttcccctggagaaaacggtgctcctggacaaatgggtcctcgtggacttccaggagaaaggggtcgtccaggcgctccaggaccagcaggtgctaggggaaacgatggtgcaacaggcgctgctggccctcctggcccaactggtcctgctggccctccaggattcccaggcgcagttggagctaaaggagaagcaggaccacagggccctaggggttctgaaggacctcagggtgttagaggtgaaccaggtcctccaggcccagctggagcagctggtccagcaggaaatccaggtgctgatggtcaacctggagctaagggcgctaatggcgcaccaggtatcgcaggcgcaccaggttttcctggcgctagaggcccaagtggtcctcaaggaccaggtggaccaccaggtccaaaaggcaattctggcgaacctggcgctccaggttctaaaggagatactggtgctaaaggcgaaccaggacctgttggtgttcagggtcctcctggtcctgctggagaagaaggaaaaagaggtgctcgtggagaaccaggaccaactggacttcctggacctcctggtgaacgtggcggacctggctcaaggggtttccctggagctgatggagtggcaggtccaaaaggccctgctggagagagaggttcaccaggtccagctggtcctaagggctcccctggtgaagcaggtagaccaggcgaagcaggattgccaggcgcaaagggattgacaggctctcctggtagtcctggcccagatggaaaaacaggcccaccaggtccagcaggacaagatggacgtccaggcccaccaggtcctcctggagcaaggggacaagctggcgttatgggttttccaggacctaaaggtgctgctggagagccaggaaaggcaggtgaaagaggagttcctggtccaccaggagcagtgggtcctgctggcaaagatggtgaagctggagcacagggccctccaggccctgctggcccagctggcgaacgtggagaacaaggcccagctggtagtccaggatttcaaggattgcctggccctgctggccctccaggagaagcaggaaaacctggagaacaaggagttcctggtgatttgggagcacctggaccttcaggagcacgtggtgaaagaggcttccctggcgagaggggtgttcaaggtccaccaggtccagcaggacctagaggtgctaatggcgctcctggcaacgatggagcaaaaggtgatgctggtgctcctggcgcacctggaagtcagggtgctcctggattgcaaggaatgcctggagagaggggtgctgctggcttgccaggcccaaagggcgataggggtgatgctggaccaaaaggtgctgatggatccccaggaaaagatggagttcgtggtcttactggcccaatcggacctccaggccctgctggcgctccaggtgataagggcgaaagtggcccaagtggacctgctggacctactggtgctagaggtgcacctggtgataggggtgaacctggaccacctggtccagctggttttgctggtcctcctggagctgatggacaacctggcgcaaagggtgaaccaggtgatgctggcgcaaagggagatgctggtccacctggacctgctggtccagcaggcccccctgggccaatcggtaatgttggagcaccaggtgctaagggagctaggggttccgctggtccacctggagcaacaggatttccaggcgctgctggtagagttggcccaccaggcccatccggaaacgcaggccctcctggtcctccaggtcctgctggcaaggagggtggcaaaggaccaaggggcgaaactggccctgctggtagacctggcgaagttggccctcctggaccaccaggtccagcaggagaaaaaggttccccaggagctgatggcccagctggtgctccaggaactccaggccctcaaggtattgctggacagagaggcgttgtgggactccctggtcaaaggggagagagaggatttccaggcttgccaggacctagtggagaacctggaaaacaaggcccatcaggcgctagtggagagcgtggacctcctggccctatgggacctcctggattggctggcccacctggcgaatcaggtcgtgaaggcgcaccaggcgcagaaggatcacctggaagagatggatcccctggtgctaaaggcgatcgtggagaaactggtccagcaggcccaccaggcgcaccaggtgcacctggcgctccaggacctgtgggaccagctggaaaatccggagataggggcgagacaggcccagcaggaccagctggacctgttggccctgctggcgctcgtggaccagcaggacctcaaggaccaaggggagataagggagaaacaggcgaacaaggcgataggggcattaagggtcataggggttttagtggcctccagggtcctcctggcccacctggatcaccaggagaacagggaccatctggtgcttccggcccagctggtccaagaggacctccaggatcagctggtgcacctggaaaagatggtcttaacggtctcccaggaccaatcggccctccaggacctagaggaagaacaggagatgctggccctgttggccctccaggacctcctggtccaccaggtccacctggtcctccatcagctggattcgatttttcatttcttccacagccaccacaagagaaagctcacgatggcggcagatattaccgtgctgatgatgctaacgttgttagggatagagatttggaagtggatacaactttgaaatccctctcccagcaaattgaaaacattagatctccagaaggttcacgtaaaaacccagctagaacatgtcgtgatttgaaaatgtgtcactccgattggaaaagtggtgaatactggattgatccaaatcagggctgtaatctcgatgctatcaaagttttctgtaacatggaaacaggcgaaacatgcgtttatcctactcaaccttccgtggctcagaaaaattggtacatctcaaaaaatcctaaagataagaggcacgtttggttcggtgaaagtatgactgatggatttcaatttgagtacggcggtcaaggtagtgatccagctgatgtggctattcaactcacatttttgcgtcttatgtccacagaggcatcacaaaacatcacttaccactgcaaaaacagtgtggcttatatggatcaacaaacaggaaaccttaagaaggctcttcttttgaagggctcaaacgagattgagattagagcagagggcaactcaaggtttacttattcagttactgttgatggctgcacttcacatactggcgcttggggtaaaacagttatcgagtataagactacaaaaacatcaagactcccaatcattgatgttgctcctctcgatgttggcgctcctgatcaagagttcggttttgatgtgggcccagtttgtttcctc

SEQ ID NO: 42 - DNA, 4167 bp, Homo sapiens
  source 1..4167: mol_type = genomic DNA
atggctcacgctcgtgttctcctcctcgctctcgctgttttggcaacagctgctgtggctgtggcttcaagttctagttttgctgattccaacccaattcgtccagttactgatagagcagcttccactttggctcaattgcttcaagaagaaactgtgaggaagggccctgctggcgataggggccctaggggcgaaaggggtccaccaggacctccaggcagggatggcgaagatggtccaactggccctcctggacctcctggccctccagggccacccggcttgggcggaaacttcgcagctcaatacgatggcaagggtgttggtcttggtcctggtcctatgggcttgatgggacctagaggcccacctggtgctgctggtgctcctggaccacagggttttcagggaccagctggcgagccaggagagccaggccaaacaggaccagctggtgcaaggggacctgctggacctcctggaaaagctggtgaagatggtcacccaggcaaaccaggacgtcctggcgaaagaggtgttgttggaccacaaggcgctaggggatttccaggtacacctggattgccaggttttaagggcattcgtggtcataacggcctcgatggattgaagggacagcctggcgcacctggcgttaagggtgaacctggagcaccaggtgaaaacggtactcctggccagactggtgcaagaggactcccaggtgaaaggggtagagttggtgctcctggacctgctggagctaggggtagtgatggtagtgttggtcctgtgggccctgctggtccaatcggttccgctggcccacctggattcccaggcgctccaggacctaaaggagaaatcggtgctgtgggtaacgcaggtcctactggtccagcaggtcctcgtggagaagtgggattgccaggactttctggtccagtgggccctccaggcaaccctggagctaacggcttgacaggagctaaaggcgcagcaggactccctggagtggctggcgcaccaggattgcctggtccaaggggtatcccaggccctgttggcgcagctggagctactggtgcacgtggacttgttggcgaaccaggccctgctggatcaaaaggcgagtctggaaataagggagaacctggttctgctggacctcaaggtcctcctggaccttctggagaagaaggaaaaaggggaccaaatggcgaggctggatcagcaggtccaccaggaccacctggacttcgtggatcccctggtagtagaggacttccaggcgctgatggtagagcaggcgttatgggaccaccaggaagtagaggagcatccggtccagcaggagttaggggtcctaacggagatgctggtagaccaggtgaaccaggtcttatgggcccaaggggcctcccaggtagtccaggaaatatcggccctgctggaaaagaaggccctgttggacttccaggtattgatggacgtcctggccctattggcccagcaggtgcaagaggagaacctggcaatattggatttccaggaccaaagggtccaacaggcgatcctggaaaaaatggagataagggtcatgctggattggcaggcgcaaggggcgctcctggtccagatggaaacaacggcgcacagggtccacctggccctcagggtgttcaaggcggaaaaggcgaacaaggcccagctggaccaccaggctttcaaggcttgccaggaccaagtggtccagcaggtgaagttggcaagccaggcgagcgtggacttcatggcgagtttggactccctggaccagcaggaccaaggggtgaaagaggccctcctggagagagtggcgctgctggaccaacaggcccaatcggtagtagaggtcctagtggacctccaggcccagatggaaataagggtgaaccaggagttgtgggcgctgttggaacagctggtccttcaggaccatcaggactcccaggcgagagaggcgctgctggcattcctggaggaaaaggtgaaaaaggcgaacctggcctccgtggcgaaatcggaaatcctggacgtgatggtgctcgtggtgcacacggcgctgtgggcgctccaggccctgctggtgctactggtgatagaggagaggctggcgcagctggcccagcaggtcctgctggcccaaggggtagtcctggtgaaagaggcgaagttggacctgctggccctaacggctttgctggccctgctggagcagcaggtcaacctggcgctaaaggtgaaaggggcggaaagggcccaaaaggtgaaaatggcgttgtgggaccaactggtccagtgggcgcagctggacctgctggtccaaatggaccaccaggaccagcaggtagtagaggagatggtggacctccaggaatgacaggttttccaggtgctgctggtagaacaggacctcctggtcctagtggtatttctggtccaccaggaccaccaggtcctgctggaaaagaaggattgaggggtccacgtggtgatcaaggaccagtgggcagaactggtgaagttggcgcagtgggaccacctggttttgctggagaaaagggcccttctggagaggcaggaacagctggtcctcctggtacacctggacctcaaggacttttgggtgcacctggtattctcggattgccaggaagtaggggcgaacgtggacttcctggcgtggcaggagcagttggagaacctggccctctcggaatcgcaggcccaccaggcgcaagaggaccaccaggagctgttggatcaccaggcgtgaatggtgcacctggcgaggctggtcgtgatggaaacccaggaaatgatggcccaccaggaagagatggtcaacctggacacaaaggcgagaggggctacccaggaaatattggcccagttggtgctgctggcgcaccaggcccacacggtccagttggaccagcaggaaaacacggtaatcgtggcgaaacaggcccttcaggcccagtgggacctgctggtgctgttggcccaagaggaccatctggacctcaaggcattagaggcgataagggagagcctggcgaaaaaggacctagaggcttgcctggttttaaaggacacaacggtctccaaggacttccaggtatcgctggtcatcatggagatcagggtgctcctggatcagtgggtccagcaggtcctagaggcccagcaggcccttccggtccagcaggaaaggatggacgtactggccaccctggaactgtgggccctgctggaattagaggtcctcaaggtcatcagggccctgctggccctccaggtccaccaggtcctccaggcccaccaggagtttcaggtggtggttacgattttggttacgatggtgatttttaccgtgctgatcaacctagaagtgctccttctctccgtcctaaagattatgaagttgatgctactttgaaatcacttaacaaccagattgagactcttctcacacctgagggatcaagaaagaatccagcacgtacatgccgtgatctcagacttagtcacccagagtggtcaagtggctattattggattgatcctaatcagggttgtacaatggaggctatcaaagtttactgtgattttccaactggagagacatgtattagggcacaacctgagaacattccagctaaaaattggtatcgttcctctaaagataagaaacatgtttggctcggagagactattaacgctggttctcagttcgagtataatgttgagggcgttacttctaaagagatggcaactcagctcgcttttatgagattgctcgctaactacgcatcccaaaacatcacttatcactgcaaaaattccattgcatatatggatgaggagacaggaaatttgaagaaagcagttattctccaaggtagtaacgatgttgagcttgtggctgagggaaatagtagattcacttacacagttttggtggatggatgctcaaagaaaactaatgagtggggcaagacaatcattgagtacaagacaaataagccttctaggctcccatttctcgatattgcacctcttgatatcggaggagctgatcacgagttttttgttgatatcggacctgtttgttttaag

SEQ ID NO: 43 - protein, 1489 aa, synthetic construct; identical to SEQ ID NO: 3

SEQ ID NO: 44 - protein, 1389 aa, synthetic construct; identical to SEQ ID NO: 6

SEQ ID NO: 45 - protein, 37 aa, synthetic construct; identical to SEQ ID NO: 9